European Patent Application EP 4 272 830 A2, published November 8, 2023. Title: Tissue Organoids. Applicant: The University of Chicago. Application EP, filed December 8, 2017. The sequence listing filed with the application follows.

SEQUENCE LISTING (67 sequences)

SEQ ID NO: 1 - DNA, 1071 bp, unidentified
  misc_feature 1..1071: note = Luciferase
  source 1..1071: mol_type = other DNA
atgccagagccagcgaagtctgctcccgccccgaaaaagggctccaagaaggcggtgactaaggcgcagaagaaaggcggcaagaagcgcaagcgcagccgcaaggagagctattccatctatgtgtacaaggttctgaagcaggtccaccctgacaccggcatttcgtccaaggccatgggcatcatgaactcgtttgtgaacgacattttcgagcgcatcgcaggtgaggcttcccgcctggcgcattacaacaagcgctcgaccatcacctccagggagatccagacggccgtgcgcctgctgctgcctggggagttggccaagcacgccgtgtccgagggtactaaggccatcaccaagtacaccagcgctaaggatccaccggtcgccaccatggcctcctccgaggacgtcatcaaggagttcatgcgcttcaaggtgcgcatggagggctccgtgaacggccacgagttcgagatcgagggcgagggcgagggccgcccctacgagggcacccagaccgccaagctgaaggtgaccaagggcggccccctgcccttcgcctgggacatcctgtcccctcagttccagtacggctccaaggcctacgtgaagcaccccgccgacatccccgactacttgaagctgtccttccccgagggcttcaagtgggagcgcgtgatgaacttcgaggacggcggcgtggtgaccgtgacccaggactcctccctgcaggacggcgagttcatctacaaggtgaagctgcgcggcaccaacttcccctccgacggccccgtaatgcagaagaagaccatgggctgggaggcctccaccgagcggatgtaccccgaggacggcgccctgaagggcgagatcaagatgaggctgaagctgaaggacggcggccactacgacgccgaggtcaagaccacctacatggccaagaagcccgtgcagctgcccggcgcctacaagaccgacatcaagctggacatcacctcccacaacgaggactacaccatcgtggaacagtacgagcgcgccgagggccgccactccaccggcgcc

SEQ ID NO: 2 - DNA, 1648 bp, unidentified
  misc_feature 1..1648: note = H2B-RFP
  source 1..1648: mol_type = other DNA
atggaagacgccaaaaacataaagaaaggcccggcgccattctatccgctggaagatggaaccgctggagagcaactgcataaggctatgaagagatacgccctggttcctggaacaattgcttttacagatgcacatatcgaggtggacatcacttacgctgagtacttcgaaatgtccgttcggttggcagaagctatgaaacgatatgggctgaatacaaatcacagaatcgtcgtatgcagtgaaaactctcttcaattctttatgccggtgttgggcgcgttatttatcggagttgcagttgcgcccgcgaacgacatttataatgaacgtgaattgctcaacagtatgggcatttcgcagcctaccgtggtgttcgtttccaaaaaggggttgcaaaaaattttgaacgtgcaaaaaaagctcccaatcatccaaaaaattattatcatggattctaaaacggattaccagggatttcagtcgatgtacacgttcgtcacatctcatctacctcccggttttaatgaatacgattttgtgccagagtccttcgatagggacaagacaattgcactgatcatgaactcctctggatctactggtctgcctaaaggtgtcgctctgcctcatagaactgcctgcgtgagattctcgcatgccagagatcctatttttggcaatcaaatcattccggatactgcgattttaagtgttgttccattccatcacggttttggaatgtttactacactcggatatttgatatgtggatttcgagtcgtcttaatgtatagatttgaagaagagctgtttctgaggagccttcaggattacaagattcaaagtgcgctgctggtgccaaccctattctccttcttcgccaaaagcactctgattgacaaatacgatttatctaatttacacgaaattgcttctggtggcgctcccctctctaaggaagtcggggaagcggttgccaagaggttccatctgccaggtatcaggcaaggatatgggctcactgagactacatcagctattctgattacacccgagggggatgataaaccgggcgcggtcggtaaagttgttccattttttgaagcgaaggttgtggatctggataccgggaaaacgctgggcgttaatcaaagaggcgaactgtgtgtgagaggtcctatgattatgtccggttatgtaaacaatccggaagcgaccaacgccttgattgacaaggatggatggctacattctggagacatagcttactgggacgaagacgaacacttcttcatcgttgaccgcctgaagtctctgattaagtacaaaggctatcaggtggctcccgctgaattggaatccatcttgctccaacaccccaacatcttcgacgcaggtgtcgcaggtcttcccgacgatgacgccggtgaacttcccgccgccgttgttgttttggagcacggaaagacgatgacggaaaaagagatcgtggattacgtcgccagtcaagtaacaaccgcgaaaaagttgcgcggaggagttgtgtttgtggacgaagtaccgaaaggtcttaccggaaaactcgacgcaagaaaaatcagagagatcctcataaaggccaagaagggcggaaagatcgccg

SEQ ID NO: 3 - DNA, 34 bp, unidentified
  misc_feature 1..34: note = gRNA expression cassette forward primer
  source 1..34: mol_type = other DNA
aaggaaaaaagcggccgctgtacaaaaaagcagg

SEQ ID NO: 4 - DNA, 24 bp, unidentified
  misc_feature 1..24: note = gRNA expression cassette reverse primer
  source 1..24: mol_type = other DNA
ggaattctaatgccaactttgtac

SEQ ID NO: 5 - DNA, 26 bp, unidentified
  misc_feature 1..26: note = Rosa26-targeting gRNA forward primer 1
  source 1..26: mol_type = other DNA
acaccggcaggcttaaaggctaaccg

SEQ ID NO: 6 - DNA, 26 bp, unidentified
  misc_feature 1..26: note = Rosa26-targeting gRNA reverse primer 1
  source 1..26: mol_type = other DNA
aaaacggttagcctttaagcctgccg

SEQ ID NO: 7 - DNA, 26 bp, unidentified
  misc_feature 1..26: note = Rosa26-targeting gRNA forward primer 2
  source 1..26: mol_type = other DNA
acaccgaggacaacgcccacacaccg

SEQ ID NO: 8 - DNA, 26 bp, unidentified
  misc_feature 1..26: note = Rosa26-targeting gRNA reverse primer 2
  source 1..26: mol_type = other DNA
aaaacggtgtgtgggcgttgtcctcg

SEQ ID NO: 9 - DNA, 26 bp, unidentified
  misc_feature 1..26: note = AAVS1-targeting gRNA forward primer 1
  source 1..26: mol_type = other DNA
acaccgtcaccaatcctgtccctagg

SEQ ID NO: 10 - DNA, 26 bp, unidentified
  misc_feature 1..26: note = AAVS1-targeting gRNA reverse primer 1
  source 1..26: mol_type = other DNA
aaaacctagggacaggattggtgacg

SEQ ID NO: 11 - DNA, 26 bp, unidentified
  misc_feature 1..26: note = AAVS1-targeting gRNA forward primer 2
  source 1..26: mol_type = other DNA
acaccgccccacagtggggccactag

SEQ ID NO: 12 - DNA, 26 bp, unidentified
  misc_feature 1..26: note = AAVS1-targeting gRNA reverse primer 2
  source 1..26: mol_type = other DNA
aaaactagtggccccactgtggggcg

SEQ ID NO: 13 - DNA, 50 bp, unidentified
  misc_feature 1..50: note = Rosa26 targeting vector forward primer 1
  source 1..50: mol_type = other DNA
gactagtgaattcggatccttaattaaggcctccgcgccgggttttggcg

SEQ ID NO: 14 - DNA, 47 bp, unidentified
  misc_feature 1..47: note = Rosa26 targeting vector reverse primer 1
  source 1..47: mol_type = other DNA
gactagtcccgggggatccaccggtcaggaacaggtggtggcggccc

SEQ ID NO: 15 - DNA, 37 bp, unidentified
  misc_feature 1..37: note = Rosa26 targeting vector forward primer 2
  source 1..37: mol_type = other DNA
cgggatccaccggtgagggcagaggaagccttctaac

SEQ ID NO: 16 - DNA, 33 bp, unidentified
  misc_feature 1..33: note = Rosa26 targeting vector reverse primer 2
  source 1..33: mol_type = other DNA
tcccccgggtacaaaatcagaaggacagggaag

SEQ ID NO: 17 - DNA, 35 bp, unidentified
  misc_feature 1..35: note = Rosa26 targeting vector forward primer 3
  source 1..35: mol_type = other DNA
ggaattcaataaaatatctttattttcattacatc

SEQ ID NO: 18 - DNA, 59 bp, unidentified
  misc_feature 1..59: note = Rosa26 targeting vector reverse primer 3
  source 1..59: mol_type = other DNA
ccttaattaaggatccacgcgtgtttaaacaccggttttacgagggtaggaagtggtac

SEQ ID NO: 19 - DNA, 37 bp, unidentified
  misc_feature 1..37: note = AAVS1 targeting vector constructed with AAVS1 hPGK-PuroR-pA donor forward primer 1
  source 1..37: mol_type = other DNA
cccaagcttctcgagttggggttgcgccttttccaag

SEQ ID NO: 20 - DNA, 31 bp, unidentified
  misc_feature 1..31: note = AAVS1 targeting vector constructed with AAVS1 hPGK-PuroR-pA donor reverse primer 1
  source 1..31: mol_type = other DNA
cccaagcttccatagagcccaccgcatcccc

SEQ ID NO: 21 - DNA, 44 bp, unidentified
  misc_feature 1..44: note = AAVS1 targeting vector constructed with AAVS1 hPGK-PuroR-pA donor forward primer 2
  source 1..44: mol_type = other DNA
cagggtctagacgccggatccggtaccctgtgccttctagttgc

SEQ ID NO: 22 - DNA, 37 bp, unidentified
  misc_feature 1..37: note = AAVS1 targeting vector constructed with AAVS1 hPGK-PuroR-pA donor reverse primer 2
  source 1..37: mol_type = other DNA
ggatccggcgtctagaccctggggagagaggtcggtg

SEQ ID NO: 23 - DNA, 37 bp, unidentified
  misc_feature 1..37: note = AAVS1 targeting vector constructed with AAVS1 hPGK-PuroR-pA donor forward primer 3
  source 1..37: mol_type = other DNA
ccgctcgagaataaaatatctttattttcattacatc

SEQ ID NO: 24 - DNA, 30 bp, unidentified
  misc_feature 1..30: note = AAVS1 targeting vector constructed with AAVS1 hPGK-PuroR-pA donor reverse primer 3
  source 1..30: mol_type = other DNA
gctctagaccaagtgacgatcacagcgatc

SEQ ID NO: 25 - DNA, 22 bp, unidentified
  misc_feature 1..22: note = Genotyping primer for CRISPR mediated knockin #1
  source 1..22: mol_type = other DNA
gagctgggaccaccttatattc

SEQ ID NO: 26 - DNA, 17 bp, unidentified
  misc_feature 1..17: note = Genotyping primer for CRISPR mediated knockin #2
  source 1..17: mol_type = other DNA
ggtgcatgacccgcaag

SEQ ID NO: 27 - DNA, 21 bp, unidentified
  misc_feature 1..21: note = Genotyping primer for CRISPR mediated knockin #3
  source 1..21: mol_type = other DNA
gagagatggctccaggaaatg

SEQ ID NO: 28 - DNA, 2391 bp, unidentified
  misc_feature 1..2391: note = CFP/YFP FRET sensor with A213R/L238S double mutant of GGBP
  source 1..2391: mol_type = other DNA
atggtgagcaagggcgaggagctgttcaccggggtggtgcccatcctggtcgagctggacggcgacgtaaacggccacaagttcagcgtgtccggcgagggcgagggcgatgccacctacggcaagctgaccctgaagttcatctgcaccaccggcaagctgcccgtgccctggcccaccctcgtgaccaccctgacctggggcgtgcagtgcttcagccgctaccccgaccacatgaagcagcacgacttcttcaagtccgccatgcccgaaggctacgtccaggagcgcaccatcttcttcaaggacgacggcaactacaagacccgcgccgaggtgaagttcgagggcgacaccctggtgaaccgcatcgagctgaagggcatcgacttcaaggaggacggcaacatcctggggcacaagctggagtacaactacatcagccacaacgtctatatcaccgccgacaagcagaagaacggcatcaaggccaacttcaagatccgccacaacatcgaggacggcagcgtgcagctcgccgaccactaccagcagaacacccccatcggcgacggccccgtgctgctgcccgacaaccactacctgagcacccagtccgccctgagcaaagaccccaacgagaagcgcgatcacatggtcctgctggagttcgtgaccgccgccgggatcactctcggcatggacgagctgtacaagggtggtaccggaggcgccgctgatactcgcattggtgtaacaatctataagtacgacgataactttatgtctgtagtgcgcaaggctattgagcaagatgcgaaagccgcgccagatgttcagctgctgatgaatgattctcagaatgaccagtccaagcagaacgatcagatcgacgtattgctggcgaaaggggtgaaggcactggcaatcaacctggttgacccggcagctgcgggtacggtgattgagaaagcgcgtgggcaaaacgtgccggtggttttcttcaacaaagaaccgtctcgtaaggcgctggatagctacgacaaagcctactacgttggcactgactccaaagagtccggcattattcaaggcgatttgattgctaaacactgggcggcgaatcagggttgggatctgaacaaagacggtcagattcagttcgtactgctgaaaggtgaaccgggccatccggatgcagaagcacgtaccacttacgtgattaaagaattgaacgataaaggcatcaaaactgaacagttacagttagataccgcaatgtgggacaccgctcaggcgaaagataagatggacgcctggctgtctggcccgaacgccaacaaaatcgaagtggttatcgccaacaacgatcggatggcaatgggcgcggttgaagcgctgaaagcacacaacaagtccagcattccggtgtttggcgtcgatgcgtcgccagaagcgctggcgctggtgaaatccggtgcactggcgggcaccgtactgaacgatgctaacaaccaggcgaaagcgacctttgatctggcgaaaaacctggccgatggtaaaggtgcggctgatggcaccaactggaaaatcgacaacaaagtggtccgcgtaccttatgttggcgtagataaagacaacctggctgaattcagcaagaaaggcgccggtaccggtggaatggtgagcaagggcgaggagctgttcaccggggtggtgcccatcctggtcgagctggacggcgacgtaaacggccacaagttcagcgtgtccggcgagggcgagggcgatgccacctacggcaagctgaccctgaagttcatctgcaccaccggcaagctgcccgtgccctggcccaccctcgtgaccaccttcggctacggcctgcagtgcttcgcccgctaccccgaccacatgaagcagcacgacttcttcaagtccgccatgcccgaaggctacgtccaggagcgcaccatcttcttcaaggacgacggcaactacaagacccgcgccgaggtgaagttcgagggcgacaccctggtgaaccgcatcgagctgaagggcatcgacttcaaggaggacggcaacatcctggggcacaagctggagtacaactacaacagccacaacgtctatatcatggccgacaagcagaagaacggcatcaaggtgaacttcaagatccgccacaacatcgaggacggcagcgtgcagctcgccgaccactaccagcagaacacccccatcggcgacggccccgtgctgctgcccgacaaccactacctgagctaccagtccgccctgagcaaagaccccaacgagaagcgcgatcacatggtcctgctggagttcgtgaccgccgccgggatcactctcggcatggacgagctg

SEQ ID NO: 29 - DNA, 4146 bp, unidentified
  misc_feature 1..4146: note = Cas9 D10A
  source 1..4146: mol_type = other DNA
gccaccatggacaagaagtactccattgggctcgctatcggcacaaacagcgtcggctgggccgtcattacggacgagtacaaggtgccgagcaaaaaattcaaagttctgggcaataccgatcgccacagcataaagaagaacctcattggcgccctcctgttcgactccggggagacggccgaagccacgcggctcaaaagaacagcacggcgcagatatacccgcagaaagaatcggatctgctacctgcaggagatctttagtaatgagatggctaaggtggatgactctttcttccataggctggaggagtcctttttggtggaggaggataaaaagcacgagcgccacccaatctttggcaatatcgtggacgaggtggcgtaccatgaaaagtacccaaccatatatcatctgaggaagaagcttgtagacagtactgataaggctgacttgcggttgatctatctcgcgctggcgcatatgatcaaatttcggggacacttcctcatcgagggggacctgaacccagacaacagcgatgtcgacaaactctttatccaactggttcagacttacaatcagcttttcgaagagaacccgatcaacgcatccggagttgacgccaaagcaatcctgagcgctaggctgtccaaatcccggcggctcgaaaacctcatcgcacagctccctggggagaagaagaacggcctgtttggtaatcttatcgccctgtcactcgggctgacccccaactttaaatctaacttcgacctggccgaagatgccaagcttcaactgagcaaagacacctacgatgatgatctcgacaatctgctggcccagatcggcgaccagtacgcagacctttttttggcggcaaagaacctgtcagacgccattctgctgagtgatattctgcgagtgaacacggagatcaccaaagctccgctgagcgctagtatgatcaagcgctatgatgagcaccaccaagacttgactttgctgaaggcccttgtcagacagcaactgcctgagaagtacaaggaaattttcttcgatcagtctaaaaatggctacgccggatacattgacggcggagcaagccaggaggaattttacaaatttattaagcccatcttggaaaaaatggacggcaccgaggagctgctggtaaagcttaacagagaagatctgttgcgcaaacagcgcactttcgacaatggaagcatcccccaccagattcacctgggcgaactgcacgctatcctcaggcggcaagaggatttctacccctttttgaaagataacagggaaaagattgagaaaatcctcacatttcggataccctactatgtaggccccctcgcccggggaaattccagattcgcgtggatgactcgcaaatcagaagagaccatcactccctggaacttcgaggaagtcgtggataagggggcctctgcccagtccttcatcgaaaggatgactaactttgataaaaatctgcctaacgaaaaggtgcttcctaaacactctctgctgtacgagtacttcacagtttataacgagctcaccaaggtcaaatacgtcacagaagggatgagaaagccagcattcctgtctggagagcagaagaaagctatcgtggacctcctcttcaagacgaaccggaaagttaccgtgaaacagctcaaagaagactatttcaaaaagattgaatgtttcgactctgttgaaatcagcggagtggaggatcgcttcaacgcatccctgggaacgtatcacgatctcctgaaaatcattaaagacaaggacttcctggacaatgaggagaacgaggacattcttgaggacattgtcctcacccttacgttgtttgaagatagggagatgattgaagaacgcttgaaaacttacgctcatctcttcgacgacaaagtcatgaaacagctcaagaggcgccgatatacaggatgggggcggctgtcaagaaaactgatcaatgggatccgagacaagcagagtggaaagacaatcctggattttcttaagtccgatggatttgccaaccggaacttcatgcagttgatccatgatgactctctcacctttaaggaggacatccagaaagcacaagtttctggccagggggacagtcttcacgagcacatcgctaatcttgcaggtagcccagctatcaaaaagggaatactgcagaccgttaaggtcgtggatgaactcgtcaaagtaatgggaaggcataagcccgagaatatcgttatcgagatggcccgagagaaccaaactacccagaagggacagaagaacagtagggaaaggatgaagaggattgaagagggtataaaagaactggggtcccaaatccttaaggaacacccagttgaaaacacccagcttcagaatgagaagctctacctgtactacctgcagaacggcagggacatgtacgtggatcaggaactggacatcaatcggctctccgactacgacgtggatcatatcgtgccccagtcttttctcaaagatgattctattgataataaagtgttgacaagatccgataaaaatagagggaagagtgataacgtcccctcagaagaagttgtcaagaaaatgaaaaattattggcggcagctgctgaacgccaaactgatcacacaacggaagttcgataatctgactaaggctgaacgaggtggcctgtctgagttggataaagccggcttcatcaaaaggcagcttgttgagacacgccagatcaccaagcacgtggcccaaattctcgattcacgcatgaacaccaagtacgatgaaaatgacaaactgattcgagaggtgaaagttattactctgaagtctaagctggtctcagatttcagaaaggactttcagttttataaggtgagagagatcaacaattaccaccatgcgcatgatgcctacctgaatgcagtggtaggcactgcacttatcaaaaaatatcccaagcttgaatctgaatttgtttacggagactataaagtgtacgatgttaggaaaatgatcgcaaagtctgagcaggaaataggcaaggccaccgctaagtacttcttttacagcaatattatgaattttttcaagaccgagattacactggccaatggagagattcggaagcgaccacttatcgaaacaaacggagaaacaggagaaatcgtgtgggacaagggtagggatttcgcgacagtccggaaggtcctgtccatgccgcaggtgaacatcgttaaaaagaccgaagtacagaccggaggcttctccaaggaaagtatcctcccgaaaaggaacagcgacaagctgatcgcacgcaaaaaagattgggaccccaagaaatacggcggattcgattctcctacagtcgcttacagtgtactggttgtggccaaagtggagaaagggaagtctaaaaaactcaaaagcgtcaaggaactgctgggcatcacaatcatggagcgatcaagcttcgaaaaaaaccccatcgactttctcgaggcgaaaggatataaagaggtcaaaaaagacctcatcattaagcttcccaagtactctctctttgagcttgaaaacggccggaaacgaatgctcgctagtgcgggcgagctgcagaaaggtaacgagctggcactgccctctaaatacgttaatttcttgtatctggccagccactatgaaaagctcaaagggtctcccgaagataatgagcagaagcagctgttcgtggaacaacacaaacactaccttgatgagatcatcgagcaaataagcgaattctccaaaagagtgatcctcgccgacgctaacctcgataaggtgctttctgcttacaataagcacagggataagcccatcagggagcaggcagaaaacattatccacttgtttactctgaccaacttgggcgcgcctgcagccttcaagtacttcgacaccaccatagacagaaagcggtacacctctacaaaggaggtcctggacgccacactgattcatcagtcaattacggggctctatgaaacaagaatcgacctctctcagctcggtggagacagcagggctgaccccaagaagaagaggaaggtgtga

SEQ ID NO: 30 - DNA, 23 bp, unidentified
  misc_feature 1..23: note = Rosa26 gRNA1
  source 1..23: mol_type = other DNA
ggcaggcttaaaggctaacctgg

SEQ ID NO: 31 - DNA, 23 bp, unidentified
  misc_feature 1..23: note = Rosa26 gRNA2
  source 1..23: mol_type = other DNA
gactggagttgcagatcacgagg

SEQ ID NO: 32 - DNA, 7695 bp, unidentified
  misc_feature 1..7695: note = Rosa26 targeting vector
  misc_feature 195: note = n is a, c, g, or t
  misc_feature 230: note = n is a, c, g, or t
  misc_feature 380: note = n is a, c, g, or t
  misc_feature 3724: note = n is a, c, g, or t
  misc_feature 4213: note = n is a, c, g, or t
  misc_feature 4297: note = n is a, c, g, or t
  misc_feature 4874: note = n is a, c, g, or t
  misc_feature 4931: note = n is a, c, g, or t
  misc_feature 4953: note = n is a, c, g, or t
  misc_feature 4993: note = n is a, c, g, or t
  misc_feature 5644: note = n is a, c, g, or t
  misc_feature 6667: note = n is a, c, g, or t
  misc_feature 6769: note = n is a, c, g, or t
  misc_feature 7147: note = n is a, c, g, or t
  misc_feature 7562: note = n is a, c, g, or t
  source 1..7695: mol_type = other DNA
ccgcggcaggccctccgagcgtggtggagccgttctgtgagacagccgggtacgagtcgtgacgctggaaggggcaagcgggtggtgggcaggaatgcggtccgccctgcagcaaccggagggggagggagaagggagcggaaaagtctccaccggacgcggccatggctcgggggggggggggcagcggaggancgcttccggccgacgtctcgtcgctgattggcttnttttcctcccgccgtgtgtgaaaacacaaatggcgtgttttggttggcgtaaggcgcctgtcagttaacggcagccggagtgcgcagccgccggcagcctcgctctgcccactgggtggggcgggaggtaggtggggtgaggcgagctgnacgtgcgggcgcggtcggcctctggcggggcgggggaggggagggagggtcagcgaaagtagctcgcgcgcgagcggccgcccaccctccccttcctctgggggagtcgttttacccgccgccggccgggcctcgtcgtctgattggctctcggggcccagaaaactggcccttgccattggctcgtgttcgtgcaagttgagtccatccgccggccagcgggggcggcgaggaggcgctcccaggttccggccctcccctcggccccgcgccgcagagtctggccgcgcgcccctgcgcaacgtggcaggaagcgcgcgctgggggcggggacgggcagtagggctgagcggctgcggggcgggtgcaagcacgtttccgacttgagttgcctcaagaggggcgtgctgagccagacctccatcgcgcactccggggagtggagggaaggagcgagggctcagttgggctgttttggaggcaggaagcacttgctctcccaaagtcgctctgagttgttatcagtaagggagctgcagtggagtaggcggggagaaggccgcacccttctccggaggggggaggggagtgttgcaatacctttctgggagttctctgctgcctcctggcttctgaggaccgccctgggcctgggagaatcccttgccccctcttcccctcgtgatctgcaactccagtctttctagtgaattcggatccttaattaaggcctccgcgccgggttttggcgcctcccgcgggcgcccccctcctcacggcgagcgctgccacgtcagacgaagggcgcagcgagcgtcctgatccttccgcccggacgctcaggacagcggcccgctgctcataagactcggccttagaaccccagtatcagcagaaggacattttaggacgggacttgggtgactctagggcactggttttctttccagagagcggaacaggcgaggaaaagtagtcccttctcggcgattctgcggagggatctccgtggggcggtgaacgccgatgattatataaggacgcgccgggtgtggcacagctagttccgtcgcagccgggatttgggtcgcggttcttgtttgtggatcgctgtgatcgtcacttggtctagacgccaccatggtgtccaagggcgaggaggtgatcaaggagttcatgcgcttcaaggtgcgcatggagggctccatgaacggccacgagttcgagatcgagggcgagggcgagggccgcccctacgagggcacccagaccgccaagctgaaggtgaccaagggcggccccctgcccttcgcctgggacatcctgtccccccagttcatgtacggctccaaggcctacgtgaagcaccccgccgacatccccgactacaagaagctgtccttccccgagggcttcaagtgggagcgcgtgatgaacttcgaggacggcggcctggtgaccgtgacccaggactcctccctgcaggacggcaccctgatctacaaggtgaagatgcgcggcaccaacttcccccccgacggccccgtgatgcagaagaagaccatgggctgggaggcctccaccgagcgcctgtacccccgcgacggcgtgctgaagggcgagatccaccaggccctgaagctgaaggacggcggccactacctggtggagttcaagaccatctacatggccaagaagcccgtgcagctgcccggctactactacgtggacaccaagctggacatcacctcccacaacgaggactacaccatcgtggagcagtacgagcgctccgagggccgccaccacctgttcctgaccggtgagggcagaggaagccttctaacatgcggtgacgtggaggagaatcccggcccttccgggatgaccgagtacaagcccacggtgcgcctcgccacccgcgacgacgtccccagggccgtacgcaccctcgccgccgcgttcgccgactaccccgccacgcgccacaccgtcgatccggaccgccacatcgagcgggtcaccgagctgcaagaactcttcctcacgcgcgtcgggctcgacatcggcaaggtgtgggtcgcggacgacggcgccgcggtggcggtctggaccacgccggagagcgtcgaagcgggggcggtgttcgccgagatcggcccgcgcatggccgagttgagcggttcccggctggccgcgcagcaacagatggaaggcctcctggcgccgcaccggcccaaggagcccgcgtggttcctggccaccgtcggcgtctcgcccgaccaccagggcaagggtctgggcagcgccgtcgtgctccccggagtggaggcggccgagcgcgccggggtgcccgccttcctggagacctccgcgccccgcaacctccccttctacgagcggctcggcttcaccgtcaccgccgacgtcgaggtgcccgaaggaccgcgcacctggtgcatgacccgcaagcccggtgcctgaatctaggtcgacctgcagaagcttgcctcgagcagcgctgctcgagagatctacgggtggcatccctgtgacccctccccagtgcctctcctggccctggaagttgccactccagtgcccaccagccttgtcctaataaaattaagttgcatcattttgtctgactaggtgtccttctataatattatggggtggaggggggtggtatggagcaaggggcaagttgggaagacaacctgtagggcctgcggggtctattgggaaccaagctggagtgcagtggcacaatcttggctcactgcaatctccgcctcctgggttcaagcgattctcctgcctcagcctcccgagttgttgggattccaggcatgcatgaccaggctcagctaatttttgtttttttggtagagacggggtttcaccatattggccaggctggtctccaactcctaatctcaggtgatctacccaccttggcctcccaaattgctgggattacaggcgtgaaccactgctcccttccctgtccttctgattttgtacccgggactagaagatgggcgggagtcttctgggcaggcttaaaggctaacctggtgtgtgggcgttgtcctgcaggggaattgaacaggtgtaaaattggagggacaagacttcccacagattttcggttttgtcgggaagttttttaataggggcaaataggaaaatggaggataggagtcatctggggtttatgcagcaaaactacaggtatattgcttgtatccgcctcggagatttccatgaggagataaagacatgtcacccgagtttatactctcctgcttagatcctactacagtatgaaatacagtgtngcgaggtagactatgtaagcagatttaatcattttaaagagcccagtacttcatatccatttctcccgctccttctgcagccttatcaaaaggtatttagaacactcattttagccccattttcatttattatactggcttatccaacccctagacagagcattggcattttccctttcctgatcttagaagtctgatgactcatgaaaccagacagattagttacatacaccacaaatcgaggctgtagctggggcctcaacactgcagttcttttataactccttagtacactttttgttgatcctttgccttgatccttaattttcagtgtctatcacctctcccgtcaggtggtgttccacatttgggcctattctcagtccagggagttttacaacaatagatgtattgagaatccaacctaaagcttaactttccactcccatgaatgcctctctcctttttctccattataactgagctatnaccattaatggtttcaggtggatgtctcctcccccaatatacctgatgtatctacatattgccaggctgatattttaagacatnaaaggtatatttcattattgagccacatggtattgattactgctactaaaattttgtcattgtacacatctgtaaaaggtggttccttttggaatgcaaagttcaggtgtttgttgtctttcctgacctaaggtcttgtgagcttgtattttttctatttaagcagtgctttctcttggactggcttgactcatggcattctacacgttattgctggtctaaatgtgattttgccaagcttcttcaggacctataattttgcttgacttgtagccaaacacaagtaaaatgattaagcaacaaatgtatttgtgaagcttggtttttaggttgttgtgttgtgtgtgcttgtgctctataataatactatccaggggctggagaggtggctcggagttcaagagcacagactgctcttccagaagtcctgagttcaattcccagcaaccacatggtggctcacaaccatctgtaatgggatctgatgccctcttctggtgtgtctgaagaccacaagtgtattcacattaaataaataatcctccttcttcttctttttttttttttaaagagaatnctgtctccagtagaattactgaagtaatgaaatactttgtgtttgttccaatatggnagccaataatcaaatactcttnagcactggaaatgtaccaaggaactattttatttaagtgnactgtggacagaggagccataactgcagacttgtgggatacagaagaccaatgcagacttaatgtcttttctcttacactaagcaataaagaaataaaaattgaacttctagtatcctatttgttaaactgctagctttactaacttttgtgcttcatctatacaaagctgaaagctaagtctgcagccattactaaacatgaaagcaagtaatgataattttggatttcaaaaatgtagggccagagtttagccagccagtggtggtgcttgcctttatgccttaatcccagcactctggaggcagagacaggcagatctctgagtttgagcccagcctggtctacacatcaagttctatctaggatagccaggaatacacacagaaaccctgttggggaggggggctctgagatttcataaaattataattgaagcattccctaatgagccactatggatgtggctaaatccgtctacctttctgatgagatttgggtattattttttctgtctctgctgttggttgggtcttttgacactgtgggctttcttaaagcctccttccctgccatgtggtctcttgtttgctactaacttcccatggcttaaatggcatggctttttgccttctaagggcagctgctgagntttgcagcctgatttccagggtggggttgggaaatctttcaaacactaaaattgtcctttaatttttttttaaaaaatgggttatataataaacctcataaaatagttatgaggagtgaggtggactaatattaatgagtccctcccctataaaagagctattaaggctttttgtcttatactaactttttttttaaatgtggtatctttagaaccaagggtcttagagttttagtatacagaaactgttgcatcgcttaatcagattttctagtttcaaatccagagaatccaaattcttcacagccaaagtcaaattaagaatttctgactttaatgttatttgctactgtgaatataaaatgatagcttttcctgaggcagggtctcactatgtatctctgcctgatctgcaacaagatatgtagactaaagttctgcctgcttttgtctcctgaatactaaggttaaaatgtagtaatacttttggaacttgcaggtcagattcttttataggggacacactaagggagcttgggtgatagttggtaaatgtgtttaagtgatgaaaacttgaattattatcaccgcaacctactttttaaaaaaaaaagccaggcctgttagagcatgctaagggatccctaggacttgctgagcacacaagagtagtacttggcaggctcctggtgagagcatatttcaaaaaacaaggcagacaaccaagaaactacagtaaggttacctgtctttaaccatctgcatatacacagggatattaaaatattccaaataatatttcattcaagttttcccccatcaaattgggacatggatttctccggtgaataggcagagttggaaactaaacaaatgttggttttgtgatttgtgaaattgttttcaagtgatagttaaagcccatgagatacagaacaaagctgctatttcgaggtctcttggttatactcagaagcacttctttgggtttccctgcactatcctgatcatgtgctaggcctnccttaggctgattgttgttcaaataacttaagtttcctgtcaggtgatgtcatatgatttcatatatcaaggcaaaacatgttatatatgttaaacatttgnacttaatgtgaaagttaggtctttgtgggttttgattttaatttcaaaacctgagctaaataagtcattttacatgtcttacatttggtgaattgtatattgtggtttgcaggcaagactctctgacctagtaaccctcctatagagcactttgctgggtcacaagtctaggagtcaagcatttcaccttgaagttgagacgttttgttagtgtatactagttatatgttggaggacatgtttatccagaagatattcaggactatttttgactgggctaaggaattgattctgattagcactgttagtgagcattgagtggcctttaggcttgaattggagtcacttgtatatctcaaataatgctggccttttttnaaaagcccttgttctttatcaccctgttttctacataatttttgttcaaagaaatacttgtttggatctccttttgacaacaatagcatgttttcaagccatattttttttcctttttttttttttttttggtttttcgagacagggtttctctgtatagccctggctgtcctggaactcactttgtagaccaggctggcctcgaactcagaaatccgcctgcctctgcctcctgagtgccgggattaaaggcgtgcaccaccacgcctggctaagttggatattttgtatataactataaccaatactaactccactgggtggatttttaattcagtcagtagtcttaagtggtctttattggcccttattaaaatctactgttcactctaacagaggctgttggactagtggnactaagcaacttcctacggatatactagcagataagggtcagggatagaaactagtctagcgttttgtatacctaccagcttatactaccttgttctgatagaaatatttaggacatctagcttatcgatccg

SEQ ID NO: 33 - DNA, 9435 bp, unidentified
  misc_feature 1..9435: note = Rosa26 targeting vector with GGBP
  misc_feature 195: note = n is a, c, g, or t
  misc_feature 230: note = n is a, c, g, or t
  misc_feature 380: note = n is a, c, g, or t
  misc_feature 5464: note = n is a, c, g, or t
  misc_feature 5953: note = n is a, c, g, or t
  misc_feature 6037: note = n is a, c, g, or t
  misc_feature 6614: note = n is a, c, g, or t
  misc_feature 6671: note = n is a, c, g, or t
  misc_feature 6693: note = n is a, c, g, or t
  misc_feature 6733: note = n is a, c, g, or t
  misc_feature 7384: note = n is a, c, g, or t
  misc_feature 8407: note = n is a, c, g, or t
  misc_feature 8509: note = n is a, c, g, or t
  misc_feature 8887: note = n is a, c, g, or t
  misc_feature 9302: note = n is a, c, g, or t
  source 1..9435: mol_type = other DNA
ccgcggcaggccctccgagcgtggtggagccgttctgtgagacagccgggtacgagtcgtgacgctggaaggggcaagcgggtggtgggcaggaatgcggtccgccctgcagcaaccggagggggagggagaagggagcggaaaagtctccaccggacgcggccatggctcgggggggggggggcagcggaggancgcttccggccgacgtctcgtcgctgattggcttnttttcctcccgccgtgtgtgaaaacacaaatggcgtgttttggttggcgtaaggcgcctgtcagttaacggcagccggagtgcgcagccgccggcagcctcgctctgcccactgggtggggcgggaggtaggtggggtgaggcgagctgnacgtgcgggcgcggtcggcctctggcggggcgggggaggggagggagggtcagcgaaagtagctcgcgcgcgagcggccgcccaccctccccttcctctgggggagtcgttttacccgccgccggccgggcctcgtcgtctgattggctctcggggcccagaaaactggcccttgccattggctcgtgttcgtgcaagttgagtccatccgccggccagcgggggcggcgaggaggcgctcccaggttccggccctcccctcggccccgcgccgcagagtctggccgcgcgcccctgcgcaacgtggcaggaagcgcgcgctgggggcggggacgggcagtagggctgagcggctgcggggcgggtgcaagcacgtttccgacttgagttgcctcaagaggggcgtgctgagccagacctccatcgcgcactccggggagtggagggaaggagcgagggctcagttgggctgttttggaggcaggaagcacttgctctcccaaagtcgctctgagttgttatcagtaagggagctgcagtggagtaggcggggagaaggccgcacccttctccggaggggggaggggagtgttgcaatacctttctgggagttctctgctgcctcctggcttctgaggaccgccctgggcctgggagaatcccttgccccctcttcccctcgtgatctgcaactccagtctttctagtgaattcggatccttaattaaggcctccgcgccgggttttggcgcctcccgcgggcgcccccctcctcacggcgagcgctgccacgtcagacgaagggcgcagcgagcgtcctgatccttccgcccggacgctcaggacagcggcccgctgctcataagactcggccttagaaccccagtatcagcagaaggacattttaggacgggacttgggtgactctagggcactggttttctttccagagagcggaacaggcgaggaaaagtagtcccttctcggcgattctgcggagggatctccgtggggcggtgaacgccgatgattatataaggacgcgccgggtgtggcacagctagttccgtcgcagccgggatttgggtcgcggttcttgtttgtggatcgctgtgatcgtcacttggtctagaggatccgggccgcatggtgagcaagggcgaggagctgttcaccggggtggtgcccatcctggtcgagctggacggcgacgtaaacggccacaagttcagcgtgtccggcgagggcgagggcgatgccacctacggcaagctgaccctgaagttcatctgcaccaccggcaagctgcccgtgccctggcccaccctcgtgaccaccctgacctggggcgtgcagtgcttcagccgctaccccgaccacatgaagcagcacgacttcttcaagtccgccatgcccgaaggctacgtccaggagcgcaccatcttcttcaaggacgacggcaactacaagacccgcgccgaggtgaagttcgagggcgacaccctggtgaaccgcatcgagctgaagggcatcgacttcaaggaggacggcaacatcctggggcacaagctggagtacaactacatcagccacaacgtctatatcaccgccgacaagcagaagaacggcatcaaggccaacttcaagatccgccacaacatcgaggacggcagcgtgcagctcgccgaccactaccagcagaacacccccatcggcgacggccccgtgctgctgcccgacaaccactacctgagcacccagtccgccctgagcaaagaccccaacgagaagcgcgatcacatggtcctgctggagttcgtgaccgccgccgggatcactctcggcatggacgagctgtacaagggtggtaccggaggcgccgctgatactcgcattggtgtaacaatctataagtacgacgataactttatgtctgtagtgcgcaaggctattgagcaagatgcgaaagccgcgccagatgttcagctgctgatgaatgattctcagaatgaccagtccaagcagaacgatcagatcgacgtattgctggcgaaaggggtgaaggcactggcaatcaacctggttgacccggcagctgcgggtacggtgattgagaaagcgcgtgggcaaaacgtgccggtggttttcttcaacaaagaaccgtctcgtaaggcgctggatagctacgacaaagcctactacgttggcactgactccaaagagtccggcattattcaaggcgatttgattgctaaacactgggcggcgaatcagggttgggatctgaacaaagacggtcagattcagttcgtactgctgaaaggtgaaccgggccatccggatgcagaagcacgtaccacttacgtgattaaagaattgaacgataaaggcatcaaaactgaacagttacagttagataccgcaatgtgggacaccgctcaggcgaaagataagatggacgcctggctgtctggcccgaacgccaacaaaatcgaagtggttatcgccaacaacgatcggatggcaatgggcgcggttgaagcgctgaaagcacacaacaagtccagcattccggtgtttggcgtcgatgcgtcgccagaagcgctggcgctggtgaaatccggtgcactggcgggcaccgtactgaacgatgctaacaaccaggcgaaagcgacctttgatctggcgaaaaacctggccgatggtaaaggtgcggctgatggcaccaactggaaaatcgacaacaaagtggtccgcgtaccttatgttggcgtagataaagacaacctggctgaattcagcaagaaaggcgccggtaccggtggaatggtgagcaagggcgaggagctgttcaccggggtggtgcccatcctggtcgagctggacggcgacgtaaacggccacaagttcagcgtgtccggcgagggcgagggcgatgccacctacggcaagctgaccctgaagttcatctgcaccaccggcaagctgcccgtgccctggcccaccctcgtgaccaccttcggctacggcctgcagtgcttcgcccgctaccccgaccacatgaagcagcacgacttcttcaagtccgccatgcccgaaggctacgtccaggagcgcaccatcttcttcaaggacgacggcaactacaagacccgcgccgaggtgaagttcgagggcgacaccctggtgaaccgcatcgagctgaagggcatcgacttcaaggaggacggcaacatcctggggcacaagctggagtacaactacaacagccacaacgtctatatcatggccgacaagcagaagaacggcatcaaggtgaacttcaagatccgccacaacatcgaggacggcagcgtgcagctcgccgaccactaccagcagaacacccccatcggcgacggccccgtgctgctgcccgacaaccactacctgagctaccagtccgccctgagcaaagaccccaacgagaagcgcgatcacatggtcctgctggagttcgtgaccgccgccgggatcactctcggcatggacgagctgtacaagggaggtggcggaagctccggtgagggcagaggaagccttctaacatgcggtgacgtggaggagaatcccggcccttccgggatgaccgagtacaagcccacggtgcgcctcgccacccgcgacgacgtccccagggccgtacgcaccctcgccgccgcgttcgccgactaccccgccacgcgccacaccgtcgatccggaccgccacatcgagcgggtcaccgagctgcaagaactcttcctcacgcgcgtcgggctcgacatcggcaaggtgtgggtcgcggacgacggcgccgcggtggcggtctggaccacgccggagagcgtcgaagcgggggcggtgttcgccgagatcggcccgcgcatggccgagttgagcggttcccggctggccgcgcagcaacagatggaaggcctcctggcgccgcaccggcccaaggagcccgcgtggttcctggccaccgtcggcgtctcgcccgaccaccagggcaagggtctgggcagcgccgtcgtgctccccggagtggaggcggccgagcgcgccggggtgcccgccttcctggagacctccgcgccccgcaacctccccttctacgagcggctcggcttcaccgtcaccgccgacgtcgaggtgcccgaaggaccgcgcacctggtgcatgacccgcaagcccggtgcctgaatctaggtcgacctgcagaagcttgcctcgagcagcgctgctcgagagatctacgggtggcatccctgtgacccctccccagtgcctctcctggccctggaagttgccactccagtgcccaccagccttgtcctaataaaattaagttgcatcattttgtctgactaggtgtccttctataatattatggggtggaggggggtggtatggagcaaggggcaagttgggaagacaacctgtagggcctgcggggtctattgggaaccaagctggagtgcagtggcacaatcttggctcactgcaatctccgcctcctgggttcaagcgattctcctgcctcagcctcccgagttgttgggattccaggcatgcatgaccaggctcagctaatttttgtttttttggtagagacggggtttcaccatattggccaggctggtctccaactcctaatctcaggtgatctacccaccttggcctcccaaattgctgggattacaggcgtgaaccactgctcccttccctgtccttctgattttgtacccgggactagaagatgggcgggagtcttctgggcaggcttaaaggctaacctggtgtgtgggcgttgtcctgcaggggaattgaacaggtgtaaaattggagggacaagacttcccacagattttcggttttgtcgggaagttttttaataggggcaaataggaaaatggaggataggagtcatctggggtttatgcagcaaaactacaggtatattgcttgtatccgcctcggagatttccatgaggagataaagacatgtcacccgagtttatactctcctgcttagatcctactacagtatgaaatacagtgtngcgaggtagactatgtaagcagatttaatcattttaaagagcccagtacttcatatccatttctcccgctccttctgcagccttatcaaaaggtatttagaacactcattttagccccattttcatttattatactggcttatccaacccctagacagagcattggcattttccctttcctgatcttagaagtctgatgactcatgaaaccagacagattagttacatacaccacaaatcgaggctgtagctggggcctcaacactgcagttcttttataactccttagtacactttttgttgatcctttgccttgatccttaattttcagtgtctatcacctctcccgtcaggtggtgttccacatttgggcctattctcagtccagggagttttacaacaatagatgtattgagaatccaacctaaagcttaactttccactcccatgaatgcctctctcctttttctccattataactgagctatnaccattaatggtttcaggtggatgtctcctcccccaatatacctgatgtatctacatattgccaggctgatattttaagacatnaaaggtatatttcattattgagccacatggtattgattactgctactaaaattttgtcattgtacacatctgtaaaaggtggttccttttggaatgcaaagttcaggtgtttgttgtctttcctgacctaaggtcttgtgagcttgtattttttctatttaagcagtgctttctcttggactggcttgactcatggcattctacacgttattgctggtctaaatgtgattttgccaagcttcttcaggacctataattttgcttgacttgtagccaaacacaagtaaaatgattaagcaacaaatgtatttgtgaagcttggtttttaggttgttgtgttgtgtgtgcttgtgctctataataatactatccaggggctggagaggtggctcggagttcaagagcacagactgctcttccagaagtcctgagttcaattcccagcaaccacatggtggctcacaaccatctgtaatgggatctgatgccctcttctggtgtgtctgaagaccacaagtgtattcacattaaataaataatcctccttcttcttctttttttttttttaaagagaatnctgtctccagtagaattactgaagtaatgaaatactttgtgtttgttccaatatggnagccaataatcaaatactcttnagcactggaaatgtaccaaggaactattttatttaagtgnactgtggacagaggagccataactgcagacttgtgggatacagaagaccaatgcagacttaatgtcttttctcttacactaagcaataaagaaataaaaattgaacttctagtatcctatttgttaaactgctagctttactaacttttgtgcttcatctatacaaagctgaaagctaagtctgcagccattactaaacatgaaagcaagtaatgataattttggatttcaaaaatgtagggccagagtttagccagccagtggtggtgcttgcctttatgccttaatcccagcactctggaggcagagacaggcagatctctgagtttgagcccagcctggtctacacatcaagttctatctaggatagccaggaatacacacagaaaccctgttggggaggggggctctgagatttcataaaattataattgaagcattccctaatgagccactatggatgtggctaaatccgtctacctttctgatgagatttgggtattattttttctgtctctgctgttggttgggtcttttgacactgtgggctttcttaaagcctccttccctgccatgtggtctcttgtttgctactaacttcccatggcttaaatggcatggctttttgccttctaagggcagctgctgagntttgcagcctgatttccagggtggggttgggaaatctttcaaacactaaaattgtcctttaatttttttttaaaaaatgggttatataataaacctcataaaatagttatgaggagtgaggtggactaatattaatgagtccctcccctataaaagagctattaaggctttttgtcttatactaactttttttttaaatgtggtatctttagaaccaagggtcttagagttttagtatacagaaactgttgcatcgcttaatcagattttctagtttcaaatccagagaatccaaattcttcacagccaaagtcaaattaagaatttctgactttaatgttatttgctactgtgaatataaaatgatagcttttcctgaggcagggtctcactatgtatctctgcctgatctgcaacaagatatgtagactaaagttctgcctgcttttgtctcctgaatactaaggttaaaatgtagtaatacttttggaacttgcaggtcagattcttttataggggacacactaagggagcttgggtgatagttggtaaatgtgtttaagtgatgaaaacttgaattattatcaccgcaacctactttttaaaaaaaaaagccaggcctgttagagcatgctaagggatccctaggacttgctgagcacacaagagtagtacttggcaggctcctggtgagagcatatttcaaaaaacaaggcagacaaccaagaaactacagtaaggttacctgtctttaaccatctgcatatacacagggatattaaaatattccaaataatatttcattcaagttttcccccatcaaattgggacatggatttctccggtgaataggcagagttggaaactaaacaaatgttggttttgtgatttgtgaaattgttttcaagtgatagttaaagcccatgagatacagaacaaagctgctatttcgaggtctcttggttatactcagaagcacttctttgggtttccctgcactatcctgatcatgtgctaggcctnccttaggctgattgttgttcaaataacttaagtttcctgtcaggtgatgtcatatgatttcatatatcaaggcaaaacatgttatatatgttaaacatttgnacttaatgtgaaagttaggtctttgtgggttttgattttaatttcaaaacctgagctaaataagtcattttacatgtcttacatttggtgaattgtatattgtggtttgcaggcaagactctctgacctagtaaccctcctatagagcactttgctgggtcacaagtctaggagtcaagcatttcaccttgaagttgagacgttttgttagtgtatactagttatatgttggaggacatgtttatccagaagatattcaggactatttttgactgggctaaggaattgattctgattagcactgttagtgagcattgagtggcctttaggcttgaattggagtcacttgtatatctcaaataatgctggccttttttnaaaagcccttgttctttatcaccctgttttctacataatttttgttcaaagaaatacttgtttggatctccttttgacaacaatagcatgttttcaagccatattttttttcctttttttttttttttttggtttttcgagacagggtttctctgtatagccctggctgtcctggaactcactttgtagaccaggctggcctcgaactcagaaatccgcctgcctctgcctcctgagtgccgggattaaaggcgtgcaccaccacgcctggctaagttggatattttgtatataactataaccaatactaactccactgggtggatttttaattcagtcagtagtcttaagtggtctttattggcccttattaaaatctactgttcactctaacagaggctgttggactagtggnactaagcaacttcctacggatatactagcagataagggtcagggatagaaactagtctagcgttttgtatacctaccagcttatactaccttgttctgatagaaatatttaggacatctagcttatcgatccg

SEQ ID NO: 34 - DNA, 747 bp, unidentified
  misc_feature 1..747: note = IgGFc (mouse)
  source 1..747: mol_type = other DNA
atgtacaggatgcaactcctgtcttgcattgcactaagtcttgcacttgtcacgaattcgatatcggccatggttagatctggttgtaagccttgcatatgtacagtcccagaagtatcatctgtcttcatcttccccccaaagcccaaggatgtgctcaccattactctgactcctaaggtcacgtgtgttgtggtagacatcagcaaggatgatcccgaggtccagttcagctggtttgtagatgatgtggaggtgcacacagctcagacgcaaccccgggaggagcagttcaacagcactttccgctcagtcagtgaacttcccatcatgcaccaggactggctcaatggcaaggagttcaaatgcagggtcaacagtgcagctttccctgcccccatcgagaaaaccatctccaaaaccaaaggcagaccgaaggctccacaggtgtacaccattccacctcccaaggagcagatggccaaggataaagtcagtctgacctgcatgataacagacttcttccctgaagacattactgtggagtggcagtggaatgggcagccagcggagaactacaagaacactcagcccatcatggacacagatggctcttacttcgtctacagcaagctcaatgtgcagaagagcaactgggaggcaggaaatactttcacctgctctgtgttacatgagggcctgcacaaccaccatactgagaagagcctctcccactctcctggtaaa

SEQ ID NO: 35 - DNA, 195 bp, unidentified
  misc_feature 1..195: note = S2-VaTx3 with signal
  source 1..195: mol_type = other DNA
atgcgccgcggccgcctgctggagatcgccctgggcttcaccgtgctgctggcctcctacacctcccacggcgccgacgccgctgaattcgagtgccgctggtacctgggcggctgcaaggaggactccgagtgctgcgagcacctgcagtgccactcctactgggagtggtgcctgtgggacggctccttctaa

SEQ ID NO: 36 - DNA, 324 bp, unidentified
  misc_feature 1..324: note = S2-DkTx with signal
  source 1..324: mol_type = other DNA
atgcgccgcggccgcctgctggagatcgccctgggcttcaccgtgctgctggcctcctacacctcccacggcgccgacgccgctgaattcggatctgactgcgccaaggagggcgaggtgtgctcctggggcaagaagtgctgcgacctggacaacttctactgccccatggagttcatcccccactgcaagaagtacaagccctacgtgcccgtgaccaccaactgcgccaaggagggcgaggtgtgcggctggggctccaagtgctgccacggcctggactgccccctggccttcatcccctactgcgagaagtaccgctaa

SEQ ID NO: 37 - DNA, 873 bp, unidentified
  misc_feature 1..873: note = VatX3 target vector cassette: signal->VaTx3->Furin->IgGFc
  source 1..873: mol_type = other DNA
atgtacaggatgcaactcctgtcttgcattgcactaagtcttgcacttgtcacgaattcgggatctgagtgccgctggtacctgggcggctgcaaggaggactccgagtgctgcgagcacctgcagtgccactcctactgggagtggtgcctgtgggacggctccttccgacggaagcgagggatatcggccatggttagatctggttgtaagccttgcatatgtacagtcccagaagtatcatctgtcttcatcttccccccaaagcccaaggatgtgctcaccattactctgactcctaaggtcacgtgtgttgtggtagacatcagcaaggatgatcccgaggtccagttcagctggtttgtagatgatgtggaggtgcacacagctcagacgcaaccccgggaggagcagttcaacagcactttccgctcagtcagtgaacttcccatcatgcaccaggactggctcaatggcaaggagttcaaatgcagggtcaacagtgcagctttccctgcccccatcgagaaaaccatctccaaaaccaaaggcagaccgaaggctccacaggtgtacaccattccacctcccaaggagcagatggccaaggataaagtcagtctgacctgcatgataacagacttcttccctgaagacattactgtggagtggcagtggaatgggcagccagcggagaactacaagaacactcagcccatcatggacacagatggctcttacttcgtctacagcaagctcaatgtgcagaagagcaactgggaggcaggaaatactttcacctgctctgtgttacatgagggcctgcacaaccaccatactgagaagagcctctcccactctcctggtaaataa

SEQ ID NO: 38 - DNA, 993 bp, unidentified
  misc_feature 1..993: note = DkTx target vector cassette: signal->DkTx->Furin->IgGFc
  source 1..993: mol_type = other DNA
atgtacaggatgcaactcctgtcttgcattgcactaagtcttgcacttgtcacgaattcgggatctgactgcgccaaggagggcgaggtgtgctcctggggcaagaagtgctgcgacctggacaacttctactgccccatggagttcatcccccactgcaagaagtacaagccctacgtgcccgtgaccaccaactgcgccaaggagggcgaggtgtgcggctggggctccaagtgctgccacggcctggactgccccctggccttcatcccctactgcgagaagtaccgccggaagcgagggatatcggccatggttagatctggttgtaagccttgcatatgtacagtcccagaagtatcatctgtcttcatcttccccccaaagcccaaggatgtgctcaccattactctgactcctaaggtcacgtgtgttgtggtagacatcagcaaggatgatcccgaggtccagttcagctggtttgtagatgatgtggaggtgcacacagctcagacgcaaccccgggaggagcagttcaacagcactttccgctcagtcagtgaacttcccatcatgcaccaggactggctcaatggcaaggagttcaaatgcagggtcaacagtgcagctttccctgcccccatcgagaaaaccatctccaaaaccaaaggcagaccgaaggctccacaggtgtacaccattccacctcccaaggagcagatggccaaggataaagtcagtctgacctgcatgataacagacttcttccctgaagacattactgtggagtggcagtggaatgggcagccagcggagaactacaagaacactcagcccatcatggacacagatggctcttacttcgtctacagcaagctcaatgtgcagaagagcaactgggaggcaggaaatactttcacctgctctgtgttacatgagggcctgcacaaccaccatactgagaagagcctctcccactctcctggtaaataa

SEQ ID NO: 39 - DNA, 681 bp, unidentified
  misc_feature 1..681: note = IgGFc (human)
  source 1..681: mol_type = other DNA
gacaaaactcacacatgcccaccgtgcccagcacctgaactcctggggggaccgtcagtcttcctcttccccccaaaacccaaggacaccctcatgatctcccggacccctgaggtcacatgcgtggtggtggacgtgagccacgaagaccctgaggtcaagttcaactggtacgtggacggcgtggaggtgcataatgccaagacaaagccgcgggaggagcagtacaacagcacgtaccgtgtggtcagcgtcctcaccgtcctgcaccaggactggctgaatggcaaggagtacaagtgcaaggtctccaacaaagccctcccagcccccatcgagaaaaccatctccaaagccaaagggcagccccgagaaccacaggtgtacaccctgcccccatcccgggaggagatgaccaagaaccaggtcagcctgacctgcctggtcaaaggcttctatcccagcgacatcgccgtggagtgggagagcaatgggcagccggagaacaactacaagaccacgcctcccgtgctggactccgacggctccttcttcctctacagcaagctcaccgtggacaagagcaggtggcagcaggggaacgtcttctcatgctccgtgatgcacgaggctctgcacaaccactacacgcagaagagcctctccctgtctccgggtaaa

SEQ ID NO: 40 - DNA, 3778 bp, unidentified
  misc_feature 1..3778: note = AAVSI targeting vector
  source 1..3778: mol_type = other DNA
tgctttctctgaccagcattctctcccctgggcctgtgccgctttctgtctgcagcttgtggcctgggtcacctctacggctggcccagatccttccctgccgcctccttcaggttccgtcttcctccactccctcttccccttgctctctgctgtgttgctgcccaaggatgctctttccggagcacttccttctcggcgctgcaccacgtgatgtcctctgagcggatcctccccgtgtctgggtcctctccgggcatctctcctccctcacccaaccccatgccgtcttcactcgctgggttcccttttccttctccttctggggcctgtgccatctctcgtttcttaggatggccttctccgacggatgtctcccttgcgtcccgcctccccttcttgtaggcctgcatcatcaccgtttttctggacaaccccaaagtaccccgtctccctggctttagccacctctccatcctcttgctttctttgcctggacaccccgttctcctgtggattcgggtcacctctcactcctttcatttgggcagctcccctaccccccttacctctctagtctgtgctagctcttccagccccctgtcatggcatcttccaggggtccgagagctcagctagtcttcttcctccaacccgggcccctatgtccacttcaggacagcatgtttgctgcctccagggatcctgtgtccccgagctgggaccaccttatattcccagggccggttaatgtggctctggttctgggtacttttatctgtcccctccaccccacagtggggcaagcttctcgagttggggttgcgccttttccaaggcagccctgggtttgcgcagggacgcggctgctctgggcgtggttccgggaaacgcagcggcgccgaccctgggtctcgcacattcttcacgtccgttcgcagcgtcacccggatcttcgccgctacccttgtgggccccccggcgacgcttcctgctccgcccctaagtcgggaaggttccttgcggttcgcggcgtgccggacgtgacaaacggaagccgcacgtctcactagtaccctcgcagacggacagcgccagggagcaatggcagcgcgccgaccgcgatgggctgtggccaatagcggctgctcagcagggcgcgccgagagcagcggccgggaaggggcggtgcgggaggcggggtgtggggcggtagtgtgggccctgttcctgcccgcgcggtgttccgcattctgcaagcctccggagcgcacgtcggcagtcggctccctcgttgaccgaatcaccgacctctctccccagggtctagacgccaccatggtgtccaagggcgaggaggtgatcaaggagttcatgcgcttcaaggtgcgcatggagggctccatgaacggccacgagttcgagatcgagggcgagggcgagggccgcccctacgagggcacccagaccgccaagctgaaggtgaccaagggcggccccctgcccttcgcctgggacatcctgtccccccagttcatgtacggctccaaggcctacgtgaagcaccccgccgacatccccgactacaagaagctgtccttccccgagggcttcaagtgggagcgcgtgatgaacttcgaggacggcggcctggtgaccgtgacccaggactcctccctgcaggacggcaccctgatctacaaggtgaagatgcgcggcaccaacttcccccccgacggccccgtgatgcagaagaagaccatgggctgggaggcctccaccgagcgcctgtacccccgcgacggcgtgctgaagggcgagatccaccaggccctgaagctgaaggacggcggccactacctggtggagttcaagaccatctacatggccaagaagcccgtgcagctgcccggctactactacgtggacaccaagctggacatcacctcccacaacgaggactacaccatcgtggagcagtacgagcgctccgagggccgccaccacctgttcctgggatccgagggcagaggaagccttctaacatgcggtgacgtggaggagaatcccggcccttccgggatgaccgagtacaagcccacggtgcgcctcgccacccgcgacgacgtccccagggccgtacgcaccctcgccgccgcgttcgccgactaccccgccacgcgccacaccgtcgatccggaccgccacatcgagcgggtcaccgagctgcaagaactcttcctcacgcgcgtcgggctcgacatcggcaaggtgtgggtcgcggacgacggcgccgcggtggcggtctggaccacgccggagagcgtcgaagcgggggcggtgttcgccgagatcggcccgcgcatggccgagttgagcggttcccggctggccgcgcagcaacagatggaaggcctcctggcgccgcaccggcccaaggagcccgcgtggttcctggccaccgtcggcgtctcgcccgaccaccagggcaagggtctgggcagcgccgtcgtgctccccggagtggaggcggccgagcgcgccggggtgcccgccttcctggagacctccgcgccccgcaacctccccttctacgagcggctcggcttcaccgtcaccgccgacgtcgaggtgcccgaaggaccgcgcacctggtgcatgacccgcaagcccggtgcctgaatctaggtcgacattctacttggtaccctgtgccttctagttgccagccatctgttgtttgcccctcccccgtgccttccttgaccctggaaggtgccactcccactgtcctttcctaataaaatgaggaaattgcatcgcattgtctgagtaggtgtcattctattctggggggtggggtggggcaggacagcaagggggaggattgggaagacaatagcaggcatgctggggatgcggtgggctctatggaagctttactagggacaggattggtgacagaaaagccccatccttaggcctcctccttcctagtctcctgatattgggtctaacccccacctcctgttaggcagattccttatctggtgacacacccccatttcctggagccatctctctccttgccagaacctctaaggtttgcttacgatggagccagagaggatcctgggagggagagcttggcagggggtgggagggaagggggggatgcgtgacctgcccggttctcagtggccaccctgcgctaccctctcccagaacctgagctgctctgacgcggctgtctggtgcgtttcactgatcctggtgctgcagcttccttacacttcccaagaggagaagcagtttggaaaaacaaaatcagaataagttggtcctgagttctaactttggctcttcacctttctagtccccaatttatattgttcctccgtgcgtcagttttacctgtgagataaggccagtagccagccccgtcctggcagggctgtggtgaggaggggggtgtccgtgtggaaaactccctttgtgagaatggtgcgtcctaggtgttcaccaggtcgtggccgcctctactccctttctctttctccatccttctttccttaaagagtccccagtgctatctgggacatattcctccgcccagagcagggtcccgcttccctaaggccctgctctgggcttctgggtttgagtccttggcaagcccaggagaggcgctcaggcttccctgtcccccttcctcgtccaccatctcatgcccctggctctcctgccccttccctacaggggttcctggctctgctct

SEQ ID NO: 41 - protein, 602 aa, unidentified
  REGION 1..602: note = Human mutant BChE
MHSKVTIICIRFLFWFLLLCMLIGKSHTEDDIIIATKNGKVRGMNLTVFGGTVTAFLGIPYAQPPLGRLRFKKPQSLTKWSDIWNATKYANSCCQNIDQSFPGFHGSEMWNPNTDLSEDCLYLNVWIPAPKPKNATVLIWIYGGGFQTGTSSLHVYDGKFLARVERVIVVSMNYRVGALGFLALPGNPEAPGNMGLFDQQLALQWVQKNIAAFGGNPKSVTLFGESSGAASVSLHLLSPGSHSLFTRAILQSGSANAPWAVTSLYEARNRTLNLAKLTGCSRENETEIIKCLRNKDPQEILLNEAFVVPYGTALGVNFGPTVDGDFLTDMPDILLELGQFKKTQILVGVNKDEGTWFLVGGAPGFSKDNNSIITRKEFQEGLKIFFPGVSEFGKESILFHYTDWVDDQRPENYREALGDVVGDYNFICPALEFTKKFSEWGNNAFFYYFEHRSSKLPWPEWMGVMHGYEIEFVFGLPLERRDNYTKAEEILSRSIVKRWANFAKYGNPNETQNNSTSWPVFKSTEQKYLTLNTESTRIMTKLRAQQCRFWTSFFPKVLEMTGNIDEAEWEWKAGFHRWNNYMMDWKNQFNDYTSKKESCVGL

SEQ ID NO: 42 - DNA, 1806 bp, unidentified
  misc_feature 1..1806: note = Nucleic acid sequence encoding the amino acid sequence of SEQ ID NO: 41
  source 1..1806: mol_type = other DNA
atgcacagcaaggtgaccatcatctgcatcaggttcctgttctggttcctgctgctgtgcatgctgatcggcaagagccacaccgaggacgacatcatcatcgccaccaagaacggcaaggtgaggggcatgaacctgaccgtgttcggcggcaccgtgaccgccttcctgggcatcccctacgcccagccccccctgggcaggctgaggttcaagaagccccagagcctgaccaagtggagcgacatctggaacgccaccaagtacgccaacagctgctgccagaacatcgaccagagcttccccggcttccacggcagcgagatgtggaaccccaacaccgacctgagcgaggactgcctgtacctgaacgtgtggatccccgcccccaagcccaagaacgccaccgtgctgatctggatctacggcggcggcttccagaccggcaccagcagcctgcacgtgtacgacggcaagttcctggccagggtggagagggtgatcgtggtgagcatgaactacagggtgggcgccctgggcttcctggccctgcccggcaaccccgaggcccccggcaacatgggcctgttcgaccagcagctggccctgcagtgggtgcagaagaacatcgccgccttcggcggcaaccccaagagcgtgaccctgttcggcgagagcagcggcgccgccagcgtgagcctgcacctgctgagccccggcagccacagcctgttcaccagggccatcctgcagagcggcagcgccaacgccccctgggccgtgaccagcctgtacgaggccaggaacaggaccctgaacctggccaagctgaccggctgcagcagggagaacgagaccgagatcatcaagtgcctgaggaacaaggacccccaggagatcctgctgaacgaggccttcgtggtgccctacggcaccgccctgggcgtgaacttcggccccaccgtggacggcgacttcctgaccgacatgcccgacatcctgctggagctgggccagttcaagaagacccagatcctggtgggcgtgaacaaggacgagggcacctggttcctggtgggcggcgcccccggcttcagcaaggacaacaacagcatcatcaccaggaaggagttccaggagggcctgaagatcttcttccccggcgtgagcgagttcggcaaggagagcatcctgttccactacaccgactgggtggacgaccagaggcccgagaactacagggaggccctgggcgacgtggtgggcgactacaacttcatctgccccgccctggagttcaccaagaagttcagcgagtggggcaacaacgccttcttctactacttcgagcacaggagcagcaagctgccctggcccgagtggatgggcgtgatgcacggctacgagatcgagttcgtgttcggcctgcccctggagaggagggacaactacaccaaggccgaggagatcctgagcaggagcatcgtgaagaggtgggccaacttcgccaagtacggcaaccccaacgagacccagaacaacagcaccagctggcccgtgttcaagagcaccgagcagaagtacctgaccctgaacaccgagagcaccaggatcatgaccaagctgagggcccagcagtgcaggttctggaccagcttcttccccaaggtgctggagatgaccggcaacatcgacgaggccgagtgggagtggaaggccggcttccacaggtggaacaactacatgatggactggaagaaccagttcaacgactacaccagcaagaaggagagctgcgtgggcctg

SEQ ID NO: 43 - protein, 603 aa, unidentified
  REGION 1..603: note = Mouse mutant BChE
MQTQHTKVTQTHFLLWILLLCMPFGKSHTEEDFIITTKTGRVRGLSMPVLGGTVTAFLGIPYAQPPLGSLRFKKPQPLNKWPDIHNATQYANSCYQNIDQAFPGFQGSEMWNPNTNLSEDCLYLNVWIPVPKPKNATVMVWIYGGGFQTGTSSLPVYDGKFLARVERVIVVSMNYRVGALGFLAFPGNPDAPGNMGLFDQQLALQWVQRNIAAFGGNPKSITIFGESSGAASVSLHLLCPQSYPLFTRAILESGSANAPWAVKHPEEARNRTLTLAKFTGCSKENEMEMIKCLRSKDPQEILRNERFVLPSDSALGINFGPTVDGDFLTDMPHTLLQLGKVKKAQILVGVNKDEGTWFLVGGAPGFSKDNDSLITRKEFQEGLNMYFPGVSRLGKEAVLFYYVDWLGEQSPEVYRDALDDVIGDYNIICPALEFTKKFAELENNAFFYFFEHRSSKLPWPEWMGVMHGYEIEFVFGLPLGRRVNYTRAEEIFSRSIMKTWANFAKYGHPNGTQGNSTMWPVFTSTEQKYLTLNTEKSKIYSKLRAPQCQFWRLFFPKVLEMTGDIDETEQEWKAGFHRWSNYMMDWQNQFNDYTSKKESCTAL

SEQ ID NO: 44 - DNA, 1809 bp, unidentified
  misc_feature 1..1809: note = Nucleic acid sequence encoding the amino acid sequence of SEQ ID NO: 43
  source 1..1809: mol_type = other DNA
atgcagacccagcacaccaaggtgacccagacccacttcctgctgtggatcctgctgctgtgcatgcccttcggcaagagccacaccgaggaggacttcatcatcaccaccaagaccggcagggtgaggggcctgagcatgcccgtgctgggcggcaccgtgaccgccttcctgggcatcccctacgcccagccccccctgggcagcctgaggttcaagaagccccagcccctgaacaagtggcccgacatccacaacgccacccagtacgccaacagctgctaccagaacatcgaccaggccttccccggcttccagggcagcgagatgtggaaccccaacaccaacctgagcgaggactgcctgtacctgaacgtgtggatccccgtgcccaagcccaagaacgccaccgtgatggtgtggatctacggcggcggcttccagaccggcaccagcagcctgcccgtgtacgacggcaagttcctggccagggtggagagggtgatcgtggtgagcatgaactacagggtgggcgccctgggcttcctggccttccccggcaaccccgacgcccccggcaacatgggcctgttcgaccagcagctggccctgcagtgggtgcagaggaacatcgccgccttcggcggcaaccccaagagcatcaccatcttcggcgagagcagcggcgccgccagcgtgagcctgcacctgctgtgcccccagagctaccccctgttcaccagggccatcctggagagcggcagcgccaacgccccctgggccgtgaagcaccccgaggaggccaggaacaggaccctgaccctggccaagttcaccggctgcagcaaggagaacgagatggagatgatcaagtgcctgaggagcaaggacccccaggagatcctgaggaacgagaggttcgtgctgcccagcgacagcgccctgggcatcaacttcggccccaccgtggacggcgacttcctgaccgacatgccccacaccctgctgcagctgggcaaggtgaagaaggcccagatcctggtgggcgtgaacaaggacgagggcacctggttcctggtgggcggcgcccccggcttcagcaaggacaacgacagcctgatcaccaggaaggagttccaggagggcctgaacatgtacttccccggcgtgagcaggctgggcaaggaggccgtgctgttctactacgtggactggctgggcgagcagagccccgaggtgtacagggacgccctggacgacgtgatcggcgactacaacatcatctgccccgccctggagttcaccaagaagttcgccgagctggagaacaacgccttcttctacttcttcgagcacaggagcagcaagctgccctggcccgagtggatgggcgtgatgcacggctacgagatcgagttcgtgttcggcctgcccctgggcaggagggtgaactacaccagggccgaggagatcttcagcaggagcatcatgaagacctgggccaacttcgccaagtacggccaccccaacggcacccagggcaacagcaccatgtggcccgtgttcaccagcaccgagcagaagtacctgaccctgaacaccgagaagagcaagatctacagcaagctgagggccccccagtgccagttctggaggctgttcttccccaaggtgctggagatgaccggcgacatcgacgagaccgagcaggagtggaaggccggcttccacaggtggagcaactacatgatggactggcagaaccagttcaacgactacaccagcaagaaggagagctgcaccgccctg

SEQ ID NO: 45 - protein, 275 aa, unidentified
  REGION 1..275: note = mGLP-1 (GLY8 mutant with IgG-Fc fusion)
MYRMQLLSCIALSLALVTNSHGEGTFTSDVSSYLEGQAAKEFIAWLVKGRGRSGCKPCICTVPEVSSVFIFPPKPKDVLTITLTPKVTCVVVDISKDDPEVQFSWFVDDVEVHTAQTQPREEQFNSTFRSVSELPIMHQDWLNGKEFKCRVNSAAFPAPIEKTISKTKGRPKAPQVYTIPPPKEQMAKDKVSLTCMITDFFPEDITVEWQWNGQPAENYKNTQPIMDTDGSYFVYSKLNVQKSNWEAGNTFTCSVLHEGLHNHHTEKSLSHSPGK

SEQ ID NO: 46 - DNA, 825 bp, unidentified
  misc_feature 1..825: note = Nucleic acid sequence encoding the amino acid sequence of SEQ ID NO: 45
  source 1..825: mol_type = other DNA
atgtacaggatgcagctgctgagctgcatcgccctgagcctggccctggtgaccaacagccacggcgagggcaccttcaccagcgacgtgagcagctacctggagggccaggccgccaaggagttcatcgcctggctggtgaagggcaggggcaggagcggctgcaagccctgcatctgcaccgtgcccgaggtgagcagcgtgttcatcttcccccccaagcccaaggacgtgctgaccatcaccctgacccccaaggtgacctgcgtggtggtggacatcagcaaggacgaccccgaggtgcagttcagctggttcgtggacgacgtggaggtgcacaccgcccagacccagcccagggaggagcagttcaacagcaccttcaggagcgtgagcgagctgcccatcatgcaccaggactggctgaacggcaaggagttcaagtgcagggtgaacagcgccgccttccccgcccccatcgagaagaccatcagcaagaccaagggcaggcccaaggccccccaggtgtacaccatccccccccccaaggagcagatggccaaggacaaggtgagcctgacctgcatgatcaccgacttcttccccgaggacatcaccgtggagtggcagtggaacggccagcccgccgagaactacaagaacacccagcccatcatggacaccgacggcagctacttcgtgtacagcaagctgaacgtgcagaagagcaactgggaggccggcaacaccttcacctgcagcgtgctgcacgagggcctgcacaaccaccacaccgagaagagcctgagccacagccccggcaag

SEQ ID NO: 47 - DNA, 36 bp, unidentified
  misc_feature 1..36: note = Primer A
  source 1..36: mol_type = other DNA
gctctagagccaccatgcagactcagcataccaagg

SEQ ID NO: 48 - DNA, 42 bp, unidentified
  misc_feature 1..42: note = Primer B
  source 1..42: mol_type = other DNA
cgggatccaccggtttagagagctgtacaagattctttcttg

SEQ ID NO: 49 - DNA, 36 bp, unidentified
  misc_feature 1..36: note = Primer C
  source 1..36: mol_type = other DNA
cccaagcttgccaccatgcatagcaaagtcacaatc

SEQ ID NO: 50 - DNA, 38 bp, unidentified
  misc_feature 1..38: note = Primer D
  source 1..38: mol_type = other DNA
acgcgtcgacttagagacccacacaactttctttcttg

SEQ ID NO: 51 - DNA, 1701 bp, unidentified
  misc_feature 1..1701: note = PAL
  source 1..1701: mol_type = other DNA
atgaagacgctgtcacaggcccagtccaagacctcctcccagcagttctccttcaccggcaactcctccgccaacgtgatcatcggcaaccagaagctgaccatcaacgacgtggcccgcgtggcccgcaacggcaccctggtgtccctgaccaacaacaccgacatcctgcagggcatccaggcctcctgcgactacatcaacaacgccgtggagtccggcgagcccatctacggcgtgacctccggcttcggcggcatggccaacgtggccatctcccgcgagcaggcctccgagctgcagaccaacctggtgtggttcctgaagaccggcgccggcaacaagctgcccctggccgacgtgcgcgccgccatgctgctgcgcgccaactcccacatgcgcggcgcctccggcatccgcctcgagctgatcaagcgcatggagatcttcctgaacgccggcgtgaccccctacgtgtacgagttcggctccatcggcgcctccggcgacctggtgcccctgtcctacatcaccggctccctgatcggcctggacccctccttcaaggtggacttcaacggcaaggagatggacgcccccaccgccctgcgccagctgaacctgtcccccctgaccctgctgcccaaggagggcctggccatgatgaacggcacctccgtgatgaccggcatcgccgccaactgcgtgtacgacacccagatcctgaccgccatcgccatgggtgtacacgctctggacatccaggccctgaacggcaccaaccagtccttccaccccttcatccacaactccaagccccaccccggccagctgtgggccgccgaccagatgatctccctcctcgccaactcccagctggtgcgcgacgagctggacggcaagcacgactaccgcgaccacgagctgatccaggaccgctactccctgcgctgcctgccccagtacctgggccccatcgtggacggcatctcccagatcgccaagcagatcgagatcgagatcaactccgtgaccgacaaccccctgatcgacgtggacaaccaggcctcctaccacggcggcaacttcctgggccagtacgtgggcatgggcatggaccacctgcgctactacatcggcctgctggccaagcacctggacgtgcagatcgccctgctggcctcccccgagttctccaacggcctgcccccctccctgctgggcaaccgcgagcgcaaggtgaacatgggcctgaagggcctgcagatctgcggtaactcgataatgcccctgctgaccttctacggcaactccatcgccgaccgcttccccacccacgccgagcagttcaaccagaacatcaactcccagggctacacctccgccaccctggcccgccgctccgtggacatcttccagaactacgtggccatcgccctgatgttcggcgttcaagctgtagacctgcgcacctacaagaagaccggccactacgacgcccgcgcctccctgtcccccgccaccgagcgcctgtactccgccgtgcgccacgtggtgggccagaagcccacctccgaccgcccctacatctggaacgacaacgagcagggcctggacgagcacatcgcccgcatctccgccgacatcgcagcaggtggcgtgatcgtgcaggccgtgcaggacatcctgccctccctgcac

SEQ ID NO: 52 - DNA, 1128 bp, unidentified
  misc_feature 1..1128: note = HSV-TK
  source 1..1128: mol_type = other DNA
atggcttcgtaccccggccatcagcacgcgtctgcgttcgaccaggctgcgcgttctcgcggccatagcaaccgacgtacggcgttgcgccctcgccggcagcaagaagccacggaagtccgcccggagcagaaaatgcccacgctactgcgggtttatatagacggtccccacgggatggggaaaaccaccaccacgcaactgctggtggccctgggttcgcgcgacgatatcgtctacgtacccgagccgatgacttactggcgggtgctgggggcttccgagacaatcgcgaacatctacaccacacaacaccgccttgaccagggtgagatatcggccggggacgcggcggtggtaatgacaagcgcccagataacaatgggcatgccttatgccgtgaccgacgccgttctggctcctcatatcgggggggaggctgggagctcacatgccccgcccccggccctcaccctcatcttcgaccgccatcccatcgccgccctcctgtgctacccggccgcgcgataccttatgggcagcatgaccccccaggccgtgctggcgttcgtggccctcatcccgccgaccttgcccggcacaaacatcgtgttgggggcccttccggaggacagacacatcgaccgcctggccaaacgccagcgccccggcgagcggcttgacctggctatgctggccgcgattcgccgcgtttacgggctgcttgccaatacggtgcggtatctgcagggcggcgggtcgtggcgggaggattggggacagctttcggggacggccgtgccgccccagggtgccgagccccagagcaacgcgggcccacgaccccatatcggggacacgttatttaccctgtttcgggcccccgagttgctggcccccaacggcgacctgtacaacgtgtttgcctgggccttggacgtcttggccaaacgcctccgtcccatgcacgtctttatcctggattacgaccaatcgcccgccggctgccgggacgccctgctgcaacttacctccgggatgatccagacccacgtcaccaccccaggctccataccgacgatctgcgacctggcgcgcacgtttgcccgggagatgggggaggctaac

SEQ ID NO: 53 - DNA, 474 bp, unidentified
  misc_feature 1..474: note = yCD
  source 1..474: mol_type = other DNA
atggtgaccggcggcatggcctccaagtgggaccagaagggcatggacatcgcctacgaggaggccgccctgggctacaaggagggcggcgtgcccatcggcggctgcctgatcaacaacaaggacggctccgtgctgggccgcggccacaacatgcgcttccagaagggctccgccaccctgcacggcgagatctccaccctggagaactgcggccgcctggagggcaaggtgtacaaggacaccaccctgtacaccaccctgtccccctgcgacatgtgcaccggcgccatcatcatgtacggcatcccccgctgcgtggtgggcgagaacgtgaacttcaagtccaagggcgagaagtacctgcagacccgcggccacgaggtggtggtggtggacgacgagcgctgcaagaagatcatgaagcagttcatcgacgagcgcccccaggactggttcgaggacatcggcgag

SEQ ID NO: 54 - DNA, 1356 bp, unidentified
  misc_feature 1..1356: note = PAH
  source 1..1356: mol_type = other DNA
atgtccactgcggtcctggaaaacccaggcttgggcaggaaactctctgactttggacaggaaacaagctatattgaagacaactgcaatcaaaatggtgccatatcactgatcttctcactcaaagaagaagttggtgcattggccaaagtattgcgcttatttgaggagaatgatgtaaacctgacccacattgaatctagaccttctcgtttaaagaaagatgagtatgaatttttcacccatttggataaacgtagcctgcctgctctgacaaacatcatcaagatcttgaggcatgacattggtgccactgtccatgagctttcacgagataagaagaaagacacagtgccctggttcccaagaaccattcaagagctggacagatttgccaatcagattctcagctatggagcggaactggatgctgaccaccctggttttaaagatcctgtgtaccgtgcaagacggaagcagtttgctgacattgcctacaactaccgccatgggcagcccatccctcgagtggaatacatggaggaagaaaagaaaacatggggcacagtgttcaagactctgaagtccttgtataaaacccatgcttgctatgagtacaatcacatttttccacttcttgaaaagtactgtggcttccatgaagataacattccccagctggaagacgtttctcaattcctgcagacttgcactggtttccgcctccgacctgtggctggcctgctttcctctcgggatttcttgggtggcctggccttccgagtcttccactgcacacagtacatcagacatggatccaagcccatgtatacccccgaacctgacatctgccatgagctgttgggacatgtgcccttgttttcagatcgcagctttgcccagttttcccaggaaattggccttgcctctctgggtgcacctgatgaatacattgaaaagctcgccacaatttactggtttactgtggagtttgggctctgcaaacaaggagactccataaaggcatatggtgctgggctcctgtcatcctttggtgaattacagtactgcttatcagagaagccaaagcttctccccctggagctggagaagacagccatccaaaattacactgtcacggagttccagcccctgtattacgtggcagagagttttaatgatgccaaggagaaagtaaggaactttgctgccacaatacctcggcccttctcagttcgctacgacccatacacccaaaggattgaggtcttggacaatacccagcagcttaagattttggctgattccattaacagtgaaattggaatcctttgcagtgccctccagaaaataaag

SEQ ID NO: 55 - DNA, 723 bp, unidentified
  misc_feature 1..723: note = GTPCH
  source 1..723: mol_type = other DNA
atggagaagccgcggggagtcaggtgcaccaatgggttctccgagcgtgaactacctcgtcctggagcaagcccacctgcagagaagtcccgacctcctgaagcaaagggcgcacagccggccgacgcctggaaggcagggcggcaccgcagcgaggaggaaaaccaggtgaacctccccaaactggcggccgcttactcgtccattctgctctcgctgggcgaggacccccagcggcaggggctgctcaagacgccctggagggcggccaccgccatgcagtacttcaccaagggataccaggagaccatctcagatgtcctgaatgatgctatatttgatgaagatcatgacgagatggtgattgtgaaggacatagatatgttctccatgtgtgagcatcaccttgttccatttgtaggaagggtccatattggctatcttcctaacaagcaagtccttggtctcagtaaacttgccaggattgtagaaatctacagtagacgactacaagttcaagagcgcctcaccaaacagattgcggtggccatcacagaagccttgcagcctgctggcgttggagtagtgattgaagcgacacacatgtgcatggtaatgcgaggcgtgcagaaaatgaacagcaagactgtcactagcaccatgctgggcgtgttccgggaagaccccaagactcgggaggagttcctcacactaatcaggagc

SEQ ID NO: 56 - DNA, 432 bp, unidentified
  misc_feature 1..432: note = PTPS
  source 1..432: mol_type = other DNA
atgagcgctgctggtgatcttcgtcgtcgtgcgcgactgtcgcgcctcgtgtccttcagcgcgagccaccggctgcacagcccatctctgagcgatgaagagaacttaagagtgtttgggaaatgcaacaatccgaatggccacgggcacaactataaagttgtggtgacagtccatggagagattgatcctgttacaggaatggttatgaatttgaccgacctcaaagaatacatggaggaggccatcatgaagcctcttgatcacaagaacctggacctggatgtgccgtactttgcggatgctgtgagcacgacagaaaatgtagctgtctacatctgggaaagcctccagaaacttcttccagtgggagctctttataaagtaaaagtgtttgaaaccgacaacaacatcgtagtctataaaggagaa

SEQ ID NO: 57 - DNA, 783 bp, unidentified
  misc_feature 1..783: note = SR (sepiapterin reductase)
  source 1..783: mol_type = other DNA
atggagggcgggctggggcgtgctgtgtgcttgctgaccggggcctcccgcggcttcggccggacgctggccccgctcctggcctcgctgctgtcgcccggctccgtgcttgtccttagcgcccgcaacgacgaggcactgcgccagctggaggccgagctgggcgccgagcggtctggcctgcgcgtggtgcgggtgcccgccgacctgggcgccgaggccggcttgcagcagctgctcggcgccctgcgcgagctcccccggcccaaggggctgcagcgactgctgcttatcaacaacgcgggctctcttggggatgtgtccaaaggcttcgtggacctgagtgactccactcaagtgaacaactactgggcactgaacttgacctccatgctctgcctgacttccagcgtcctgaaggccttcccggacagtcctggcctcaacagaaccgtggttaacatctcgtccctctgtgccctgcaacctttcaaaggctgggcgctgtactgtgcaggaaaggctgctcgtgatatgctgttccaggtcctggcgctggaggaacctaatgtgagggtgctgaactatgccccaggtcctctggacacagacatgcagcagttggcccgggagacctccgtggacccagacatgcgaaaagggctgcaggagctgaaggcaaaggggaagctggtggattgcaaggtgtcagcccagaaactgctgagcttactggaaaaggacgagttcaagtctggagcccacgtggacttctatgacaaa

SEQ ID NO: 58 - DNA, 4413 bp, unidentified
  misc_feature 1..4413: note = Factor VIII minus B
  source 1..4413: mol_type = other DNA
atgcaaatagagctctccacctgcttctttctgtgccttttgcgattctgctttagtgccaccagaagatactacctgggtgcagtggaactgtcatgggactatatgcaaagtgatctcggtgagctgcctgtggacgcaagatttcctcctagagtgccaaaatcttttccattcaacacctcagtcgtgtacaaaaagactctgtttgtagaattcacggatcaccttttcaacatcgctaagccaaggccaccctggatgggtctgctaggtcctaccatccaggctgaggtttatgatacagtggtcattacacttaagaacatggcttcccatcctgtcagtcttcatgctgttggtgtatcctactggaaagcttctgagggagctgaatatgatgatcagaccagtcaaagggagaaagaagatgataaagtcttccctggtggaagccatacatatgtctggcaggtcctgaaagagaatggtccaatggcctctgacccactgtgccttacctactcatatctttctcatgtggacctggtaaaagacttgaattcaggcctcattggagccctactagtatgtagagaagggagtctggccaaggaaaagacacagaccttgcacaaatttatactactttttgctgtatttgatgaagggaaaagttggcactcagaaacaaagaactccttgatgcaggatagggatgctgcatctgctcgggcctggcctaaaatgcacacagtcaatggttatgtaaacaggtctctgccaggtctgattggatgccacaggaaatcagtctattggcatgtgattggaatgggcaccactcctgaagtgcactcaatattcctcgaaggtcacacatttcttgtgaggaaccatcgccaggcgtccttggaaatctcgccaataactttccttactgctcaaacactcttgatggaccttggacagtttctactgttttgtcatatctcttcccaccaacatgatggcatggaagcttatgtcaaagtagacagctgtccagaggaaccccaactacgaatgaaaaataatgaagaagcggaagactatgatgatgatcttactgattctgaaatggatgtggtcaggtttgatgatgacaactctccttcctttatccaaattcgctcagttgccaagaagcatcctaaaacttgggtacattacattgctgctgaagaggaggactgggactatgctcccttagtcctcgcccccgatgacagaagttataaaagtcaatatttgaacaatggccctcagcggattggtaggaagtacaaaaaagtccgatttatggcatacacagatgaaacctttaagactcgtgaagctattcagcatgaatcaggaatcttgggacctttactttatggggaagttggagacacactgttgattatatttaagaatcaagcaagcagaccatataacatctaccctcacggaatcactgatgtccgtcctttgtattcaaggagattaccaaaaggtgtaaaacatttgaaggattttccaattctgccaggagaaatattcaaatataaatggacagtgactgtagaagatgggccaactaaatcagatcctcggtgcctgacccgctattactctagtttcgttaatatggagagagatctagcttcaggactcattggccctctcctcatctgctacaaagaatctgtagatcaaagaggaaaccagataatgtcagacaagaggaatgtcatcctgttttctgtatttgatgagaaccgaagctggtacctcacagagaatatacaacgctttctccccaatccagctggagtgcagcttgaggatccagagttccaagcctccaacatcatgcacagcatcaatggctatgtttttgatagtttgcagttgtcagtttgtttgcatgaggtggcatactggtacattctaagcattggagcacagactgacttcctttctgtcttcttctctggatataccttcaaacacaaaatggtctatgaagacacactcaccctattcccattctcaggagaaactgtcttcatgtcgatggaaaacccaggtctatggattctggggtgccacaactcagactttcggaacagaggcatgaccgccttactgaaggtttctagttgtgacaagaacactggtgattattacgaggacagttatgaagatatttcagcatacttgctgagtaaaaacaatgccattgaaccaagaagcttctcccagaattcaagacaccctagcactaggcaaaagcaatttaatgccaccccaccagtcttgaaacgccatcaacgggaaataactcgtactactcttcagtcagatcaagaggaaattgactatgatgataccatatcagttgaaatgaagaaggaagattttgacatttatgatgaggatgaaaatcagagcccccgcagctttcaaaagaaaacacgacactattttattgctgcagtggagaggctctgggattatgggatgagtagctccccacatgttctaagaaacagggctcagagtggcagtgtccctcagttcaagaaagttgttttccaggaatttactgatggctcctttactcagcccttataccgtggagaactaaatgaacatttgggactcctggggccatatataagagcagaagttgaagataatatcatggtaactttcagaaatcaggcctctcgtccctattccttctattctagccttatttcttatgaggaagatcagaggcaaggagcagaacctagaaaaaactttgtcaagcctaatgaaaccaaaacttacttttggaaagtgcaacatcatatggcacccactaaagatgagtttgactgcaaagcctgggcttatttctctgatgttgacctggaaaaagatgtgcactcaggcctgattggaccccttctggtctgccacactaacacactgaaccctgctcatgggagacaagtgacagtacaggaatttgctctgtttttcaccatctttgatgagaccaaaagctggtacttcactgaaaatatggaaagaaactgcagggctccctgcaatatccagatggaagatcccacttttaaagagaattatcgcttccatgcaatcaatggctacataatggatacactacctggcttagtaatggctcaggatcaaaggattcgatggtatctgctcagcatgggcagcaatgaaaacatccattctattcatttcagtggacatgtgttcactgtacgaaaaaaagaggagtataaaatggcactgtacaatctctatccaggtgtttttgagacagtggaaatgttaccatccaaagctggaatttggcgggtggaatgccttattggcgagcatctacatgctgggatgagcacactttttctggtgtacagcaataagtgtcagactcccctgggaatggcttctggacacattagagattttcagattacagcttcaggacaatatggacagtgggccccaaagctggccagacttcattattccggatcaatcaatgcctggagcaccaaggagcccttttcttggatcaaggtggatctgttggcaccaatgattattcacggcatcaagacccagggtgcccgtcagaagttctccagcctctacatctctcagtttatcatcatgtatagtcttgatgggaagaagtggcagacttatcgaggaaattccactggaaccttaatggtcttctttggcaatgtggattcatctgggataaaacacaatatttttaaccctccaattattgctcgatacatccgtttgcacccaactcattatagcattcgcagcactcttcgcatggagttgatgggctgtgatttaaatagttgcagcatgccattgggaatggagagtaaagcaatatcagatgcacagattactgcttcatcctactttaccaatatgtttgccacctggtctccttcaaaagctcgacttcacctccaagggaggagtaatgcctggagacctcaggtgaataatccaaaagagtggctgcaagtggacttccagaagacaatgaaagtcacaggagtaactactcagggagtaaaatctctgcttaccagcatgtatgtgaaggagttcctcatctccagcagtcaagatggccatcagtggactctcttttttcagaatggcaaagtaaaggtttttcagggaaatcaagactccttcacacctgtggtgaactctctagacccaccgttactgactcgctaccttcgaattcacccccagagttgggtgcaccagattgccctgaggatggaggttctgggctgcgaggcacaggacctctac

SEQ ID NO: 59 - DNA, 7053 bp, unidentified
  misc_feature 1..7053: note = Factor VIII
  source 1..7053: mol_type = other DNA
atgcaaatagagctctccacctgcttctttctgtgccttttgcgattctgctttagtgccaccagaagatactacctgggtgcagtggaactgtcatgggactatatgcaaagtgatctcggtgagctgcctgtggacgcaagatttcctcctagagtgccaaaatcttttccattcaacacctcagtcgtgtacaaaaagactctgtttgtagaattcacggatcaccttttcaacatcgctaagccaaggccaccctggatgggtctgctaggtcctaccatccaggctgaggtttatgatacagtggtcattacacttaagaacatggcttcccatcctgtcagtcttcatgctgttggtgtatcctactggaaagcttctgagggagctgaatatgatgatcagaccagtcaaagggagaaagaagatgataaagtcttccctggtggaagccatacatatgtctggcaggtcctgaaagagaatggtccaatggcctctgacccactgtgccttacctactcatatctttctcatgtggacctggtaaaagacttgaattcaggcctcattggagccctactagtatgtagagaagggagtctggccaaggaaaagacacagaccttgcacaaatttatactactttttgctgtatttgatgaagggaaaagttggcactcagaaacaaagaactccttgatgcaggatagggatgctgcatctgctcgggcctggcctaaaatgcacacagtcaatggttatgtaaacaggtctctgccaggtctgattggatgccacaggaaatcagtctattggcatgtgattggaatgggcaccactcctgaagtgcactcaatattcctcgaaggtcacacatttcttgtgaggaaccatcgccaggcgtccttggaaatctcgccaataactttccttactgctcaaacactcttgatggaccttggacagtttctactgttttgtcatatctcttcccaccaacatgatggcatggaagcttatgtcaaagtagacagctgtccagaggaaccccaactacgaatgaaaaataatgaagaagcggaagactatgatgatgatcttactgattctgaaatggatgtggtcaggtttgatgatgacaactctccttcctttatccaaattcgctcagttgccaagaagcatcctaaaacttgggtacattacattgctgctgaagaggaggactgggactatgctcccttagtcctcgcccccgatgacagaagttataaaagtcaatatttgaacaatggccctcagcggattggtaggaagtacaaaaaagtccgatttatggcatacacagatgaaacctttaagactcgtgaagctattcagcatgaatcaggaatcttgggacctttactttatggggaagttggagacacactgttgattatatttaagaatcaagcaagcagaccatataacatctaccctcacggaatcactgatgtccgtcctttgtattcaaggagattaccaaaaggtgtaaaacatttgaaggattttccaattctgccaggagaaatattcaaatataaatggacagtgactgtagaagatgggccaactaaatcagatcctcggtgcctgacccgctattactctagtttcgttaatatggagagagatctagcttcaggactcattggccctctcctcatctgctacaaagaatctgtagatcaaagaggaaaccagataatgtcagacaagaggaatgtcatcctgttttctgtatttgatgagaaccgaagctggtacctcacagagaatatacaacgctttctccccaatccagctggagtgcagcttgaggatccagagttccaagcctccaacatcatgcacagcatcaatggctatgtttttgatagtttgcagttgtcagtttgtttgcatgaggtggcatactggtacattctaagcattggagcacagactgacttcctttctgtcttcttctctggatataccttcaaacacaaaatggtctatgaagacacactcaccctattcccattctcaggagaaactgtcttcatgtcgatggaaaacccaggtctatggattctggggtgccacaactcagactttcggaacagaggcatgaccgccttactgaaggtttctagttgtgacaagaacactggtgattattacgaggacagttatgaagatatttcagcatacttgctgagtaaaaacaatgccattgaaccaagaagcttctcccagaattcaagacaccctagcactaggcaaaagcaatttaatgccaccacaattccagaaaatgacatagagaagactgacccttggtttgcacacagaacacctatgcctaaaatacaaaatgtctcctctagtgatttgttgatgctcttgcgacagagtcctactccacatgggctatccttatctgatctccaagaagccaaatatgagactttttctgatgatccatcacctggagcaatagacagtaataacagcctgtctgaaatgacacacttcaggccacagctccatcacagtggggacatggtatttacccctgagtcaggcctccaattaagattaaatgagaaactggggacaactgcagcaacagagttgaagaaacttgatttcaaagtttctagtacatcaaataatctgatttcaacaattccatcagacaatttggcagcaggtactgataatacaagttccttaggacccccaagtatgccagttcattatgatagtcaattagataccactctatttggcaaaaagtcatctccccttactgagtctggtggacctctgagcttgagtgaagaaaataatgattcaaagttgttagaatcaggtttaatgaatagccaagaaagttcatggggaaaaaatgtatcgtcaacagagagtggtaggttatttaaagggaaaagagctcatggacctgctttgttgactaaagataatgccttattcaaagttagcatctctttgttaaagacaaacaaaacttccaataattcagcaactaatagaaagactcacattgatggcccatcattattaattgagaatagtccatcagtctggcaaaatatattagaaagtgacactgagtttaaaaaagtgacacctttgattcatgacagaatgcttatggacaaaaatgctacagctttgaggctaaatcatatgtcaaataaaactacttcatcaaaaaacatggaaatggtccaacagaaaaaagagggccccattccaccagatgcacaaaatccagatatgtcgttctttaagatgctattcttgccagaatcagcaaggtggatacaaaggactcatggaaagaactctctgaactctgggcaaggccccagtccaaagcaattagtatccttaggaccagaaaaatctgtggaaggtcagaatttcttgtctgagaaaaacaaagtggtagtaggaaagggtgaatttacaaaggacgtaggactcaaagagatggtttttccaagcagcagaaacctatttcttactaacttggataatttacatgaaaataatacacacaatcaagaaaaaaaaattcaggaagaaatagaaaagaaggaaacattaatccaagagaatgtagttttgcctcagatacatacagtgactggcactaagaatttcatgaagaaccttttcttactgagcactaggcaaaatgtagaaggttcatatgacggggcatatgctccagtacttcaagattttaggtcattaaatgattcaacaaatagaacaaagaaacacacagctcatttctcaaaaaaaggggaggaagaaaacttggaaggcttgggaaatcaaaccaagcaaattgtagagaaatatgcatgcaccacaaggatatctcctaatacaagccagcagaattttgtcacgcaacgtagtaagagagctttgaaacaattcagactcccactagaagaaacagaacttgaaaaaaggataattgtggatgacacctcaacccagtggtccaaaaacatgaaacatttgaccccgagcaccctcacacagatagactacaatgagaaggagaaaggggccattactcagtctcccttatcagattgccttacgaggagtcatagcatccctcaagcaaatagatctccattacccattgcaaaggtatcatcatttccatctattagacctatatatctgaccagggtcctattccaagacaactcttctcatcttccagcagcatcttatagaaagaaagattctggggtccaagaaagcagtcatttcttacaaggagccaaaaaaaataacctttctttagccattctaaccttggagatgactggtgatcaaagagaggttggctccctggggacaagtgccacaaattcagtcacatacaagaaagttgagaacactgttctcccgaaaccagacttgcccaaaacatctggcaaagttgaattgcttccaaaagttcacatttatcagaaggacctattccctacggaaactagcaatgggtctcctggccatctggatctcgtggaagggagccttcttcagggaacagagggagcgattaagtggaatgaagcaaacagacctggaaaagttccctttctgagagtagcaacagaaagctctgcaaagactccctccaagctattggatcctcttgcttgggataaccactatggtactcagataccaaaagaagagtggaaatcccaagagaagtcaccagaaaaaacagcttttaagaaaaaggataccattttgtccctgaacgcttgtgaaagcaatcatgcaatagcagcaataaatgagggacaaaataagcccgaaatagaagtcacctgggcaaagcaaggtaggactgaaaggctgtgctctcaaaacccaccagtcttgaaacgccatcaacgggaaataactcgtactactcttcagtcagatcaagaggaaattgactatgatgataccatatcagttgaaatgaagaaggaagattttgacatttatgatgaggatgaaaatcagagcccccgcagctttcaaaagaaaacacgacactattttattgctgcagtggagaggctctgggattatgggatgagtagctccccacatgttctaagaaacagggctcagagtggcagtgtccctcagttcaagaaagttgttttccaggaatttactgatggctcctttactcagcccttataccgtggagaactaaatgaacatttgggactcctggggccatatataagagcagaagttgaagataatatcatggtaactttcagaaatcaggcctctcgtccctattccttctattctagccttatttcttatgaggaagatcagaggcaaggagcagaacctagaaaaaactttgtcaagcctaatgaaaccaaaacttacttttggaaagtgcaacatcatatggcacccactaaagatgagtttgactgcaaagcctgggcttatttctctgatgttgacctggaaaaagatgtgcactcaggcctgattggaccccttctggtctgccacactaacacactgaaccctgctcatgggagacaagtgacagtacaggaatttgctctgtttttcaccatctttgatgagaccaaaagctggtacttcactgaaaatatggaaagaaactgcagggctccctgcaatatccagatggaagatcccacttttaaagagaattatcgcttccatgcaatcaatggctacataatggatacactacctggcttagtaatggctcaggatcaaaggattcgatggtatctgctcagcatgggcagcaatgaaaacatccattctattcatttcagtggacatgtgttcactgtacgaaaaaaagaggagtataaaatggcactgtacaatctctatccaggtgtttttgagacagtggaaatgttaccatccaaagctggaatttggcgggtggaatgccttattggcgagcatctacatgctgggatgagcacactttttctggtgtacagcaataagtgtcagactcccctgggaatggcttctggacacattagagattttcagattacagcttcaggacaatatggacagtgggccccaaagctggccagacttcattattccggatcaatcaatgcctggagcaccaaggagcccttttcttggatcaaggtggatctgttggcaccaatgattattcacggcatcaagacccagggtgcccgtcagaagttctccagcctctacatctctcagtttatcatcatgtatagtcttgatgggaagaagtggcagacttatcgaggaaattccactggaaccttaatggtcttctttggcaatgtggattcatctgggataaaacacaatatttttaaccctccaattattgctcgatacatccgtttgcacccaactcattatagcattcgcagcactcttcgcatggagttgatgggctgtgatttaaatagttgcagcatgccattgggaatggagagtaaagcaatatcagatgcacagattactgcttcatcctactttaccaatatgtttgccacctggtctccttcaaaagctcgacttcacctccaagggaggagtaatgcctggagacctcaggtgaataatccaaaagagtggctgcaagtggacttccagaagacaatgaaagtcacaggagtaactactcagggagtaaaatctctgcttaccagcatgtatgtgaaggagttcctcatctccagcagtcaagatggccatcagtggactctcttttttcagaatggcaaagtaaaggtttttcagggaaatcaagactccttcacacctgtggtgaactctctagacccaccgttactgactcgctaccttcgaattcacccccagagttgggtgcaccagattgccctgaggatggaggttctgggctgcgaggcacaggacctctac

SEQ ID NO: 60 - DNA, 1827 bp, unidentified
  misc_feature 1..1827: note = Albumin
  source 1..1827: mol_type = other DNA
atgaagtgggtaacctttatttcccttctttttctctttagctcggcttattccaggggtgtgtttcgtcgagatgcacacaagagtgaggttgctcatcggtttaaagatttgggagaagaaaatttcaaagccttggtgttgattgcctttgctcagtatcttcagcagtgtccatttgaagatcatgtaaaattagtgaatgaagtaactgaatttgcaaaaacatgtgttgctgatgagtcagctgaaaattgtgacaaatcacttcataccctttttggagacaaattatgcacagttgcaactcttcgtgaaacctatggtgaaatggctgactgctgtgcaaaacaagaacctgagagaaatgaatgcttcttgcaacacaaagatgacaacccaaacctcccccgattggtgagaccagaggttgatgtgatgtgcactgcttttcatgacaatgaagagacatttttgaaaaaatacttatatgaaattgccagaagacatccttacttttatgccccggaactccttttctttgctaaaaggtataaagctgcttttacagaatgttgccaagctgctgataaagctgcctgcctgttgccaaagctcgatgaacttcgggatgaagggaaggcttcgtctgccaaacagagactcaagtgtgccagtctccaaaaatttggagaaagagctttcaaagcatgggcagtagctcgcctgagccagagatttcccaaagctgagtttgcagaagtttccaagttagtgacagatcttaccaaagtccacacggaatgctgccatggagatctgcttgaatgtgctgatgacagggcggaccttgccaagtatatctgtgaaaatcaagattcgatctccagtaaactgaaggaatgctgtgaaaaacctctgttggaaaaatcccactgcattgccgaagtggaaaatgatgagatgcctgctgacttgccttcattagctgctgattttgttgaaagtaaggatgtttgcaaaaactatgctgaggcaaaggatgtcttcctgggcatgtttttgtatgaatatgcaagaaggcatcctgattactctgtcgtgctgctgctgagacttgccaagacatatgaaaccactctagagaagtgctgtgccgctgcagatcctcatgaatgctatgccaaagtgttcgatgaatttaaacctcttgtggaagagcctcagaatttaatcaaacaaaattgtgagctttttgagcagcttggagagtacaaattccagaatgcgctattagttcgttacaccaagaaagtaccccaagtgtcaactccaactcttgtagaggtctcaagaaacctaggaaaagtgggcagcaaatgttgtaaacatcctgaagcaaaaagaatgccctgtgcagaagactatctatccgtggtcctgaaccagttatgtgtgttgcatgagaaaacgccagtaagtgacagagtcaccaaatgctgcacagaatccttggtgaacaggcgaccatgcttttcagctctggaagtcgatgaaacatacgttcccaaagagtttaatgctgaaacattcaccttccatgcagatatatgcacactttctgagaaggagagacaaatcaagaaacaaactgcacttgttgagctcgtgaaacacaagcccaaggcaacaaaagagcaactgaaagctgttatggatgatttcgcagcttttgtagagaagtgctgcaaggctgacgataaggagacctgctttgccgaggagggtaaaaaacttgttgctgcaagtcaagctgccttaggctta

SEQ ID NO: 61 - DNA, 1389 bp, unidentified
  misc_feature 1..1389: note = Factor IX
  source 1..1389: mol_type = other DNA
gccaccatgcagcgcgtgaacatgatcatggcagaatcaccaggcctcatcaccatctgccttttaggatatctactcagtgctgaatgtacagtttttcttgatcatgaaaacgccaacaaaattctgaatcggccaaagaggtataattcaggtaaattggaagagtttgttcaagggaaccttgagagagaatgtatggaagaaaagtgtagttttgaagaagcacgagaagtttttgaaaacactgaaagaacaactgaattttggaagcagtatgttgatggagatcagtgtgagtccaatccatgtttaaatggcggcagttgcaaggatgacattaattcctatgaatgttggtgtccctttggatttgaaggaaagaactgtgaattagatgtaacatgtaacattaagaatggcagatgcgagcagttttgtaaaaatagtgctgataacaaggtggtttgctcctgtactgagggatatcgacttgcagaaaaccagaagtcctgtgaaccagcagtgccatttccatgtggaagagtttctgtttcacaaacttctaagctcacccgtgctgagactgtttttcctgatgtggactatgtaaattctactgaagctgaaaccattttggataacatcactcaaagcacccaatcatttaatgacttcactcgggttgttggtggagaagatgccaaaccaggtcaattcccttggcaggttgttttgaatggtaaagttgatgcattctgtggaggctctatcgttaatgaaaaatggattgtaactgctgcccactgtgttgaaactggtgttaaaattacagttgtcgcaggtgaacataatattgaggagacagaacatacagagcaaaagcgaaatgtgattcgaattattcctcaccacaactacaatgcagctattaataagtacaaccatgacattgcccttctggaactggacgaacccttagtgctaaacagctacgttacacctatttgcattgctgacaaggaatacacgaacatcttcctcaaatttggatctggctatgtaagtggctggggaagagtcttccacaaagggagatcagctttagttcttcagtaccttagagttccacttgttgaccgagccacatgtcttcgatctacaaagttcaccatctataacaacatgttctgtgctggcttccatgaaggaggtagagattcatgtcaaggagatagtgggggaccccatgttactgaagtggaagggaccagtttcttaactggaattattagctggggtgaagagtgtgcaatgaaaggcaaatatggaatatataccaaggtatcccggtatgtcaactggattaaggaaaaaacaaagctcact

SEQ ID NO: 62 - DNA, 432 bp, unidentified
  misc_feature 1..432: note = H-FABP
  source 1..432: mol_type = other DNA
atggtggacgctttcctgggcacctggaagctagtggacagcaagaatttcgatgactacatgaagtcactcgctcatatactcataaccttccccctaccctcaggtgtgggttttgctaccaggcaggtggccagcatgaccaagcctaccacaatcatcgaaaagaatggggacattctcaccctaaaaacacacagcaccttcaagaacacagagatcagctttaagttgggggtggagttcgatgagacaacagcagatgacaggaaggtcaagtccattgtgacactggatggagggaaacttgttcacctgcagaaatgggacgggcaagagaccacacttgtgcgggagctaattgatggaaaactcatcctgacactcacccacggcactgcagtttgcactcgcacttatgagaaagaggca

SEQ ID NO: 63 - DNA, 462 bp, unidentified
  misc_feature 1..462: note = Myocardial myoglobin
  source 1..462: mol_type = other DNA
atggggctcagcgacggggaatggcagttggtgctgaacgtctgggggaaggtggaggctgacatcccaggccatgggcaggaagtcctcatcaggctctttaagggtcacccagagactctggagaagtttgacaagttcaagcacctgaagtcagaggacgagatgaaggcgtctgaggacttaaagaagcatggtgccaccgtgctcaccgccctgggtggcatccttaagaagaaggggcatcatgaggcagagattaagcccctggcacagtcgcatgccaccaagcacaagatccccgtgaagtacctggagttcatctcggaatgcatcatccaggttctgcagagcaagcatcccggggactttggtgctgatgcccagggggccatgaacaaggccctggagctgttccggaaggacatggcctccaactacaaggagctgggcttccagggc

SEQ ID NO: 64 - DNA, 1293 bp, unidentified
  misc_feature 1..1293: note = GFAP
  source 1..1293: mol_type = other DNA
atggagaggagacgcatcacctccgctgctcgccgctcctacgtctcctcaggggagatgatggtggggggcctggctcctggccgccgtctgggtcctggcacccgcctctccctggctcgaatgccccctccactcccgacccgggtggatttctccctggctggggcactcaatgctggcttcaaggagacccgggccagtgagcgggcagagatgatggagctcaatgaccgctttgccagctacatcgagaaggttcgcttcctggaacagcaaaacaaggcgctggctgctgagctgaaccagctgcgggccaaggagcccaccaagctggcagacgtctaccaggctgagctgcgagagctgcggctgcggctcgatcaactcaccgccaacagcgcccggctggaggttgagagggacaatctggcacaggacctggccactgtgaggcagaagctccaggatgaaaccaacctgaggctggaagccgagaacaacctggctgcctatagacaggaagcagatgaagccaccctggcccgtctggatctggagaggaagattgagtcgctggaggaggagatccggttcttgaggaagatccacgaggaggaggttcgggaactccaggagcagctggcccgacagcaggtccatgtggagcttgacgtggccaagccagacctcaccgcagccctgaaagagatccgcacgcagtatgaggcaatggcgtccagcaacatgcatgaagccgaagagtggtaccgctccaagtttgcagacctgacagacgctgctgcccgcaacgcggagctgctccgccaggccaagcacgaagccaacgactaccggcgccagttgcagtccttgacctgcgacctggagtctctgcgcggcacgaacgagtccctggagaggcagatgcgcgagcaggaggagcggcacgtgcgggaggcggccagttatcaggaggcgctggcgcggctggaggaagaggggcagagcctcaaggacgagatggcccgccacttgcaggagtaccaggacctgctcaatgtcaagctggccctggacatcgagatcgccacctacaggaagctgctagagggcgaggagaaccggatcaccattcccgtgcagaccttctccaacctgcagattcgagggggcaaaagcaccaaagacggggaaaatcacaaggtcacaagatatctcaaaagcctcacaatacgagttataccaatacaggctcaccagattgtaaatggaacgccgccggctcgcggt

SEQ ID NO: 65 - DNA, 276 bp, unidentified
  misc_feature 1..276: note = S100B
  source 1..276: mol_type = other DNA
atgtctgagctggagaaggccatggtggccctcatcgacgttttccaccaatattctggaagggagggagacaagcacaagctgaagaaatccgaactgaaggagctcatcaacaatgagctttcccatttcttagaggaaatcaaagagcaggaggttgtggacaaagtcatggaaacactggacaatgatggagacggcgaatgtgacttccaggaattcatggcctttgttgccatggttactactgcctgccacgagttctttgaacatgag

SEQ ID NO: 66 - DNA, 1069 bp, unidentified
  misc_feature 1..1069: note = PYY (Homo sapiens)
  source 1..1069: mol_type = other DNA
gcccctggaggaactgaacccactatcggtcatggggccgagactaaatgtggcgggttgtctttaatctgctgccaagaggaaactcattcaggcaagttcagccctttatgaggaattcccctgtggtcacattccaattcctggacctgctgccaccctcagaactgcatgctccttcttcagactttctaagaatgactcaggtcattggtggagtgaagtcaagatttccaactcagtcacctgaagagatggagataccattcatggagctggaggtccctggagatttgggaattcagataacaagctaagataaggagtttgcctacctctgtcctagagcgaagcctgagccttgggcgcgcagcacaccacaagtatctgttactgtgttttgcagaagcttcaggcggggatataagccccacaaggaaagcgctgagcagaggaggcctcagcttgacctgcggcagtgcagcccttgggacttccctcgccttccacctcctgctcgtctgcttcacaagctatcgctatggtgttcgtgcgcaggccgtggcccgccttgaccacagtgcttctggccctgctcgtctgcctaggggcgctggtcgacgcctaccccatcaaacccgaggctcccggcgaagacgcctcgccggaggagctgaaccgctactacgcctccctgcgccactacctcaacctggtcacccggcagcggtatgggaaaagagacggcccggacacgcttctttccaaaacgttcttccccgacggcgaggaccgccccgtcaggtcgcggtcggagggcccagacctgtggtgaggacccctgaggcctcctgggagatctgccaaccacgcccacgtcatttgcatacgcactcccgaccccagaaacccggattctgcctcccgacggcggcgtctgggcagggttcgggtgcggccctccgcccgcgtctcggtgcccccgccccctgggctggagggctgtgtgtggtccttccctggtcccaaaataaagagcaaattccacagaaacggaaaaaaaaaaaaa

SEQ ID NO: 67 - DNA, 3670 bp, unidentified
  misc_feature 1..3670: note = TIMP2 (Homo sapiens)
  source 1..3670: mol_type = other DNA
cgcagcaaacacatccgtagaaggcagcgcggccgccgagaaccgcagcgccgctcgcccgccgccccccaccccgccgccccgcccggcgaattgcgccccgcgcccctcccctcgcgcccccgagacaaagaggagagaaagtttgcgcggccgagcggggcaggtgaggagggtgagccgcgcgggaggggcccgcctcggccccggctcagcccccgcccgcgcccccagcccgccgccgcgagcagcgcccggaccccccagcggcggcccccgcccgcccagccccccggcccgccatgggcgccgcggcccgcaccctgcggctggcgctcggcctcctgctgctggcgacgctgcttcgcccggccgacgcctgcagctgctccccggtgcacccgcaacaggcgttttgcaatgcagatgtagtgatcagggccaaagcggtcagtgagaaggaagtggactctggaaacgacatttatggcaaccctatcaagaggatccagtatgagatcaagcagataaagatgttcaaagggcctgagaaggatatagagtttatctacacggccccctcctcggcagtgtgtggggtctcgctggacgttggaggaaagaaggaatatctcattgcaggaaaggccgagggggacggcaagatgcacatcaccctctgtgacttcatcgtgccctgggacaccctgagcaccacccagaagaagagcctgaaccacaggtaccagatgggctgcgagtgcaagatcacgcgctgccccatgatcccgtgctacatctcctccccggacgagtgcctctggatggactgggtcacagagaagaacatcaacgggcaccaggccaagttcttcgcctgcatcaagagaagtgacggctcctgtgcgtggtaccgcggcgcggcgccccccaagcaggagtttctcgacatcgaggacccataagcaggcctccaacgcccctgtggccaactgcaaaaaaagcctccaagggtttcgactggtccagctctgacatcccttcctggaaacagcatgaataaaacactcatcccatgggtccaaattaatatgattctgctccccccttctccttttagacatggttgtgggtctggagggagacgtgggtccaaggtcctcatcccatcctccctctgccaggcactatgtgtctggggcttcgatccttgggtgcaggcagggctgggacacgcggcttccctcccagtccctgccttggcaccgtcacagatgccaagcaggcagcacttagggatctcccagctgggttagggcagggcctggaaatgtgcattttgcagaaacttttgagggtcgttgcaagactgtgtagcaggcctaccaggtccctttcatcttgagagggacatggcccttgttttctgcagcttccacgcctctgcactccctgcccctggcaagtgctcccatcgccccggtgcccaccatgagctcccagcacctgactccccccacatccaagggcagcctggaaccagtggctagttcttgaaggagccccatcaatcctattaatcctcagaattccagtgggagcctccctctgagccttgtagaaatgggagcgagaaaccccagctgagctgcgttccagcctcagctgagtctttttggtctgcacccacccccccacccccccccccccgcccacatgctccccagcttgcaggaggaatcggtgaggtcctgtcctgaggctgctgtccggggccggtggctgccctcaaggtcccttccctagctgctgcggttgccattgcttcttgcctgttctggcatcaggcacctggattgagttgcacagctttgctttatccgggcttgtgtgcagggcccggctgggctccccatctgcacatcctgaggacagaaaaagctgggtcttgctgtgccctcccaggcttagtgttccctccctcaaagactgacagccatcgttctgcacggggctttctgcatgtgacgccagctaagcatagtaagaagtccagcctaggaagggaaggattttggaggtaggtggctttggtgacacactcacttctttctcagcctccaggacactatggcctgttttaagagacatcttatttttctaaaggtgaattctcagatgataggtgaacctgagttgcagatataccaacttctgcttgtatttcttaaatgacaaagattacctagctaagaaacttcctagggaactagggaacctatgtgttccctcagtgtggtttcctgaagccagtgatatgggggttaggataggaagaactttctcggtaatgataaggagaatctcttgtttcctcccacctgtgttgtaaagataaactgacgatatacaggcacattatgtaaacatacacacgcaatgaaaccgaagcttggcggcctgggcgtggtcttgcaaaatgcttccaaagccaccttagcctgttctattcagcggcaaccccaaagcacctgttaagactcctgacccccaagtggcatgcagcccccatgcccaccgggacctggtcagcacagatcttgatgacttccctttctagggcagactgggagggtatccaggaatcggcccctgccccacgggcgttttcatgctgtacagtgacctaaagttggtaagatgtcataatggaccagtccatgtgatttcagtatatacaactccaccagacccctccaacccatataacaccccacccctgttcgcttcctgtatggtgatatcatatgtaacatttactcctgtttctgctgattgtttttttaatgttttggtttgtttttgacatcagctgtaatcattcctgtgctgtgttttttattacccttggtaggtattagacttgcacttttttaaaaaaaggtttctgcatcgtggaagcatttgacccagagtggaacgcgtggcctatgcaggtggattccttcaggtctttcctttggttctttgagcatctttgctttcattcgtctcccgtctttggttctccagttcaaattattgcaaagtaaaggatctttgagtaggttcggtctgaaaggtgtggcctttatatttgatccacacacgttggtcttttaaccgtgctgagcagaaaacaaaacaggttaagaagagccgggtggcagctgacagaggaagccgctcaaataccttcacaataaatagtggcaatatatatatagtttaagaaggctctccatttggcatcgtttaatttatatgttatgttctaagcacagctctcttctcctattttcatcctgcaagcaactcaaaatatttaaaataaagtttacattgtagttattttcaaatctttgcttgataagtattaagaaatattggacttgctgccgtaatttaaagctctgttgattttgtttccgtttggatttttgggggaggggagcactgtgtttatgctggaatatgaagtctgagaccttccggtgctgggaacacacaagagttgttgaaagttgacaagcagactgcgcatgtctctgatgctttgtatcattcttgagcaatcgctcggtccgtggacaataaacagtattatcaaagagaaaaaaaaaaaaaaaaa